European Patent Application EP 4 397 686 A1, published July 10, 2024. Title: 抗GPRC5D抗原结合蛋白及其用途. Applicant: 原启生物科技（上海）有限责任公司. The sequence listing filed with the application follows.

SEQUENCE LISTING (220 sequences)

SEQ ID NO: 1 - DNA, 1038 bp, synthetic construct
  misc_feature 1..1038: note = GPRC5D nucleotide sequence
  source 1..1038: mol_type = other DNA
atgtacaaggactgcatcgagtccactggagactattttcttctctgtgacgccgaggggccatggggcatcattctggagtccctggccatacttggcatcgtggtcacaattctgctactcttagcatttctcttcctcatgcgaaagatccaagactgcagccagtggaatgtcctccccacccagctcctcttcctcctgagtgtcctggggctcttcggactcgcttttgccttcatcatcgagctcaatcaacaaactgcccccgtacgctactttctctttggggttctctttgctctctgtttctcatgcctcttagctcatgcctccaatctagtgaagctggttcggggttgtgtctccttctcctggacgacaattctgtgcattgctattggttgcagtctgttgcaaatcattattgccactgagtatgtgactctcatcatgaccagaggtatgatgtttgtgaatatgacaccctgccagctcaatgtggactttgttgtactcctggtctatgtcctcttcctgatggccctcacattcttcgtctccaaagccaccttctgtggcccgtgtgagaactggaagcagcatggaaggctcatctttatcactgtgctcttctccatcatcatctgggtggtgtggatctccatgctcctgagaggcaacccgcagttccagcgacagccccagtgggacgacccggtcgtctgcattgctctggtcaccaacgcatgggttttcctgctgctgtacatcgtccctgagctctgcattctctacagatcgtgtagacaggagtgccctttacaaggcaatgcctgccccgtcacagcctaccaacacagcttccaagtggagaaccaggagctctccagagcccgagacagtgatggagctgaggaggatgtagcattaacttcatatggtactcccattcagccgcagactgttgatcccacacaagagtgtttcatcccacaggctaaactaagcccccagcaagatgcaggaggagtatga

SEQ ID NO: 2 - protein, 345 aa, synthetic construct
  REGION 1..345: note = GPRC5D amino acid sequence
MYKDCIESTGDYFLLCDAEGPWGIILESLAILGIVVTILLLLAFLFLMRKIQDCSQWNVLPTQLLFLLSVLGLFGLAFAFIIELNQQTAPVRYFLFGVLFALCFSCLLAHASNLVKLVRGCVSFSWTTILCIAIGCSLLQIIIATEYVTLIMTRGMMFVNMTPCQLNVDFVVLLVYVLFLMALTFFVSKATFCGPCENWKQHGRLIFITVLFSIIIWVVWISMLLRGNPQFQRQPQWDDPVVCIALVTNAWVFLLLYIVPELCILYRSCRQECPLQGNACPVTAYQHSFQVENQELSRARDSDGAEEDVALTSYGTPIQPQTVDPTQECFIPQAKLSPQQDAGGV

SEQ ID NO: 3 - DNA, 363 bp, synthetic construct
  misc_feature 1..363: note = 3B5 VHH nucleotide sequence
  source 1..363: mol_type = other DNA
gaggtgcagctggtggagagcggtggtggtctcgtgcagcccggcggtagtctgcgcctcagctgtgccgccagcggttttatctttagccgctatggcatgggctggtttcgccaagcccccggcaaaggtcgcgaactggtggccgccattaactggagcgatggcaccacctattacccagatagcgtggaaggccgcttcaccatcagccgcgataacgccaagcgcatggtgtatctgcagatgaacagtctgcgcgccgaggacaccgccgtgtattattgtgccgccgatcgccgcctgcgcagccagaccggctacgattactggggccaaggcacccaagtgaccgtgagcagc

SEQ ID NO: 4 - protein, 121 aa, synthetic construct
  REGION 1..121: note = 3B5 VHH amino acid sequence
EVQLVESGGGLVQPGGSLRLSCAASGFIFSRYGMGWFRQAPGKGRELVAAINWSDGTTYYPDSVEGRFTISRDNAKRMVYLQMNSLRAEDTAVYYCAADRRLRSQTGYDYWGQGTQVTVSS

SEQ ID NO: 5 - DNA, 372 bp, synthetic construct
  misc_feature 1..372: note = 3E7 VHH nucleotide sequence
  source 1..372: mol_type = other DNA
gaggtgcagctggtggagagcggtggtggtctcgtgcagcccggcggtagtctgcgcctcagctgtgccgccagcggtcgcatctttagccgcgatgccatgggctggtttcgccaagcccccggcaaaggtcgcgaactggtggccgccattaacagcagcggtggcaacacctattacccagatagcgtggaaggccgcttcaccatcagccgcgataacgccaagcgcatggtgtatctgcagatgaacagtctgcgcgccgaggacaccgccgtgtattattgtgccgcccgcggcgtgcgctggaccagcaccaccgcctatggctacaattactggggccaaggcacccaagtgaccgtgagcagc

SEQ ID NO: 6 - protein, 124 aa, synthetic construct
  REGION 1..124: note = 3E7 VHH amino acid sequence
EVQLVESGGGLVQPGGSLRLSCAASGRIFSRDAMGWFRQAPGKGRELVAAINSSGGNTYYPDSVEGRFTISRDNAKRMVYLQMNSLRAEDTAVYYCAARGVRWTSTTAYGYNYWGQGTQVTVSS

SEQ ID NO: 7 - DNA, 372 bp, synthetic construct
  misc_feature 1..372: note = 4A2 VHH nucleotide sequence
  source 1..372: mol_type = other DNA
gaggtgcagctggtggagagcggtggtggtctcgtgcagcccggcggtagtctgcgcctcagctgtgccgccagcggttttatctttagccgctatgatatgggctggtttcgccaagcccccggcaaaggtcgcgaactggtggccgtgattacctggggcggtggcagcacctattacccagatagcgtggaaggccgcttcaccatcagccgcgataacgccaagcgcatggtgtatctgcagatgaacagtctgcgcgccgaggacaccgccgtgtattattgtgccgcccgcagcgccagcgcctatcgcaccggccgcctggaatacaattactggggccaaggcacccaagtgaccgtgagcagc

SEQ ID NO: 8 - protein, 124 aa, synthetic construct
  REGION 1..124: note = 4A2 VHH amino acid sequence
EVQLVESGGGLVQPGGSLRLSCAASGFIFSRYDMGWFRQAPGKGRELVAVITWGGGSTYYPDSVEGRFTISRDNAKRMVYLQMNSLRAEDTAVYYCAARSASAYRTGRLEYNYWGQGTQVTVSS

SEQ ID NO: 9 - DNA, 363 bp, synthetic construct
  misc_feature 1..363: note = 4B3 VHH nucleotide sequence
  source 1..363: mol_type = other DNA
gaggtgcagctggtggagagcggtggtggtctcgtgcagcccggcggtagtctgcgcctcagctgtgccgccagcggtctgatctttagccgctatgtgatgggctggtttcgccaagcccccggcaaaggtcgcgaactggtggcctttattaacagcagcggtggcagcaccaactacccagatagcgtggaaggccgcttcaccatcagccgcgataacgccaagcgcatggtgtatctgcagatgaacagtctgcgcgccgaggacaccgccgtgtattattgtgccgccagcagccgcaccagcaccacccgcggctacaattactggggccaaggcacccaagtgaccgtgagcagc

SEQ ID NO: 10 - protein, 121 aa, synthetic construct
  REGION 1..121: note = 4B3 VHH amino acid sequence
EVQLVESGGGLVQPGGSLRLSCAASGLIFSRYVMGWFRQAPGKGRELVAFINSSGGSTNYPDSVEGRFTISRDNAKRMVYLQMNSLRAEDTAVYYCAASSRTSTTRGYNYWGQGTQVTVSS

SEQ ID NO: 11 - DNA, 372 bp, synthetic construct
  misc_feature 1..372: note = 3E9 VHH nucleotide sequence
  source 1..372: mol_type = other DNA
gaggtgcagctggtggagagcggtggtggtctcgtgcagcccggcggtagtctgcgcctcagctgtgccgccagcggttttatctttagccgctatgatatgggctggtttcgccaagcccccggcaaaggtcgcgaactggtggccgccattaactggggcgatagcagcacctattacccagatagcgtggaaggccgcttcaccatcagccgcgataacgccaagcgcatggtgtatctgcagatgaacagtctgcgcgccgaggacaccgccgtgtattattgtgccgcccgccgctattatagctattatccaagcagcggcggctacaattactggggccaaggcacccaagtgaccgtgagcagc

SEQ ID NO: 12 - protein, 124 aa, synthetic construct
  REGION 1..124: note = 3E9 VHH amino acid sequence
EVQLVESGGGLVQPGGSLRLSCAASGFIFSRYDMGWFRQAPGKGRELVAAINWGDSSTYYPDSVEGRFTISRDNAKRMVYLQMNSLRAEDTAVYYCAARRYYSYYPSSGGYNYWGQGTQVTVSS

SEQ ID NO: 13 - DNA, 363 bp, synthetic construct
  misc_feature 1..363: note = 3F5 VHH nucleotide sequence
  source 1..363: mol_type = other DNA
gaggtgcagctggtggagagcggtggtggtctcgtgcagcccggcggtagtctgcgcctcagctgtgccgccagcggttttatccttagccgctatgtgatgggctggtttcgccaagcccccggcaaaggtcgcgaactggtggcctttattacctggagcgatggcagcacctattacccagatagcgtggaaggccgcttcaccatcagccgcgataacgccaagcgcatggtgtatctgcagatgaacagtctgcgcgccgaggacaccgccgtgtattattgtgccgccaaaagccgcacctatcgcggcggcctgtacgattactggggccaaggcacccaagtgaccgtgagcagc

SEQ ID NO: 14 - protein, 121 aa, synthetic construct
  REGION 1..121: note = 3F5 VHH amino acid sequence
EVQLVESGGGLVQPGGSLRLSCAASGFILSRYVMGWFRQAPGKGRELVAFITWSDGSTYYPDSVEGRFTISRDNAKRMVYLQMNSLRAEDTAVYYCAAKSRTYRGGLYDYWGQGTQVTVSS

SEQ ID NO: 15 - DNA, 372 bp, synthetic construct
  misc_feature 1..372: note = 3G4 VHH nucleotide sequence
  source 1..372: mol_type = other DNA
gaggtgcagctggtggagagcggtggtggtctcgtgcagcccggcggtagtctgcgcctcagctgtgccgccagcggtagcatctttagcacctatcgcatgggctggtttcgccaagcccccggcaaaggtcgcgaactggtggccggcattagcccaggcggtagcgatacctattacccagatagcgtggaaggccgcttcaccatcagccgcgataacgccaagcgcatggtgtatctgcagatgaacagtctgcgcgccgaggacaccgccgtgtattattgtgccgccaccccaggccgctttgccctgctgagcccacgcggctacaattactggggccaaggcacccaagtgaccgtgagcagc

SEQ ID NO: 16 - protein, 124 aa, synthetic construct
  REGION 1..124: note = 3G4 VHH amino acid sequence
EVQLVESGGGLVQPGGSLRLSCAASGSIFSTYRMGWFRQAPGKGRELVAGISPGGSDTYYPDSVEGRFTISRDNAKRMVYLQMNSLRAEDTAVYYCAATPGRFALLSPRGYNYWGQGTQVTVSS

SEQ ID NO: 17 - DNA, 384 bp, synthetic construct
  misc_feature 1..384: note = 4A4 VHH nucleotide sequence
  source 1..384: mol_type = other DNA
gaggtgcagctggtggagagcggtggtggtctcgtgcagcccggcggtagtctgcgcctcagctgtgccgccagcggttttatctttagccgcaatgccatgggctggtttcgccaagcccccggcaaaggtcgcgaactggtggccgccattaactggagcggtagcagcaccttttacccagatagcgtggaaggccgcttcaccatcagccgcgataacgccaagcgcatggtgtatctgcagatgaacagtctgcgcgccgaggacaccgccgtgtattattgtgccgccggcagccgcaccaacaccggcaccgattggagccgcacccgctatacctacaattactggggccaaggcacccaagtgaccgtgagcagc

SEQ ID NO: 18 - protein, 128 aa, synthetic construct
  REGION 1..128: note = 4A4 VHH amino acid sequence
EVQLVESGGGLVQPGGSLRLSCAASGFIFSRNAMGWFRQAPGKGRELVAAINWSGSSTFYPDSVEGRFTISRDNAKRMVYLQMNSLRAEDTAVYYCAAGSRTNTGTDWSRTRYTYNYWGQGTQVTVSS

SEQ ID NO: 19 - DNA, 363 bp, synthetic construct
  misc_feature 1..363: note = 4E12 VHH nucleotide sequence
  source 1..363: mol_type = other DNA
gaggtgcagctggtggagagcggtggtggtctcgtgcagcccggcggtagtctgcgcctcagctgtgccgccagcggttttatctttagccgcaatagcatgggctggtttcgccaagcccccggcaaaggtcgcgaactggtggcctttattagctggcgcgatggcagcacctattacccagatagcgtggaaggccgcttcaccatcagccgcgataacgccaagcgcatggtgtatctgcagatgaacagtctgcgcgccgaggacaccgccgtgtattattgtgccgcctttcgcggctggaacaacggccgcaactacaattactggggccaaggcacccaagtgaccgtgagcagc

SEQ ID NO: 20 - protein, 121 aa, synthetic construct
  REGION 1..121: note = 4E12 VHH amino acid sequence
EVQLVESGGGLVQPGGSLRLSCAASGFIFSRNSMGWFRQAPGKGRELVAFISWRDGSTYYPDSVEGRFTISRDNAKRMVYLQMNSLRAEDTAVYYCAAFRGWNNGRNYNYWGQGTQVTVSS

SEQ ID NO: 21 - DNA, 363 bp, synthetic construct
  misc_feature 1..363: note = 4F10 VHH nucleotide sequence
  source 1..363: mol_type = other DNA
gaggtgcagctggtggagagcggtggtggtctcgtgcagcccggcggtagtctgcgcctcagctgtgccgccagcggttttatctttagcctgaatgccatgggctggtttcgccaagcccccggcaaaggtcgcgaactggtggccgccattagcccaggcgatggcaccacctattacccagatagcgtggaaggccgcttcaccatcagccgcgataacgccaagcgcatggtgtatctgcagatgaacagtctgcgcgccgaggacaccgccgtgtattattgtgccgcccgccgccgcagcctgagcggctatggctacaattactggggccaaggcacccaagtgaccgtgagcagc

SEQ ID NO: 22 - protein, 121 aa, synthetic construct
  REGION 1..121: note = 4F10 VHH amino acid sequence
EVQLVESGGGLVQPGGSLRLSCAASGFIFSLNAMGWFRQAPGKGRELVAAISPGDGTTYYPDSVEGRFTISRDNAKRMVYLQMNSLRAEDTAVYYCAARRRSLSGYGYNYWGQGTQVTVSS

SEQ ID NO: 23 - DNA, 363 bp, synthetic construct
  misc_feature 1..363: note = 505A1 VHH nucleotide sequence
  source 1..363: mol_type = other DNA
gaggtgcagctggtggagagcggtggtggtctcgtgcagcccggcggtagtctgcgcctcagctgtgccgccagcggttatatctttagccgctataacatgggctggtttcgccaagcccccggcaaaggtcgcgaactggtggccgccattagcgccggcggtagcagcacctattacccagatagcgtggaaggccgcttcaccatcagccgcgataacgccaagcgcatggtgtatctgcagatgaacagtctgcgcgccgaggacaccgccgtgtattattgtgccgcccgccgccgccgcgccaccgatagcccatacgattactggggccaaggcacccaagtgaccgtgagcagc

SEQ ID NO: 24 - protein, 121 aa, synthetic construct
  REGION 1..121: note = 505A1 VHH amino acid sequence
EVQLVESGGGLVQPGGSLRLSCAASGYIFSRYNMGWFRQAPGKGRELVAAISAGGSSTYYPDSVEGRFTISRDNAKRMVYLQMNSLRAEDTAVYYCAARRRRATDSPYDYWGQGTQVTVSS

SEQ ID NO: 25 - DNA, 372 bp, synthetic construct
  misc_feature 1..372: note = 505A3 VHH nucleotide sequence
  source 1..372: mol_type = other DNA
gaggtgcagctggtggagagcggtggtggtctcgtgcagcccggcggtagtctgcgcctcagctgtgccgccagcggttttatctttagccgctatagcatgggctggtttcgccaagcccccggcaaaggtcgcgaactggtggccggcattaactggcgcgatagcagcacctattacccagatagcgtggaaggccgcttcaccatcagccgcgataacgccaagcgcatggtgtatctgcagatgaacagtctgcgcgccgaggacaccgccgtgtattattgtgccgcctttgcccgcagcccacgcaccagcaccgaatatctgtacgattactggggccaaggcacccaagtgaccgtgagcagc

SEQ ID NO: 26 - protein, 124 aa, synthetic construct
  REGION 1..124: note = 505A3 VHH amino acid sequence
EVQLVESGGGLVQPGGSLRLSCAASGFIFSRYSMGWFRQAPGKGRELVAGINWRDSSTYYPDSVEGRFTISRDNAKRMVYLQMNSLRAEDTAVYYCAAFARSPRTSTEYLYDYWGQGTQVTVSS

SEQ ID NO: 27 - DNA, 372 bp, synthetic construct
  misc_feature 1..372: note = 505A11 VHH nucleotide sequence
  source 1..372: mol_type = other DNA
gaggtgcagctggtggagagcggtggtggtctcgtgcagcccggcggtagtctgcgcctcagctgtgccgccagcggtatcatctttagccgctatgtgatgggctggtttcgccaagcccccggcaaaggtcgcgaactggtggccgccattaccagcggcggtggcagcacccactacccagatagcgtggaaggccgcttcaccatcagccgcgataacgccaagcgcatggtgtatctgcagatgaacagtctgcgcgccgaggacaccgccgtgtattattgtgccgccggcccacgcccaaactatggccagcgctataacacctacaattactggggccaaggcacccaagtgaccgtgagcagc

SEQ ID NO: 28 - protein, 124 aa, synthetic construct
  REGION 1..124: note = 505A11 VHH amino acid sequence
EVQLVESGGGLVQPGGSLRLSCAASGIIFSRYVMGWFRQAPGKGRELVAAITSGGGSTHYPDSVEGRFTISRDNAKRMVYLQMNSLRAEDTAVYYCAAGPRPNYGQRYNTYNYWGQGTQVTVSS

SEQ ID NO: 29 - DNA, 384 bp, synthetic construct
  misc_feature 1..384: note = 505B12 VHH nucleotide sequence
  source 1..384: mol_type = other DNA
gaggtgcagctggtggagagcggtggtggtctcgtgcagcccggcggtagtctgcgcctcagctgtgccgccagcggttttatctttagccgctatatcatgggctggtttcgccaagcccccggcaaaggtcgcgaactggtggccggcattaacgccggcggtggcagcacctattacccagatagcgtggaaggccgcttcaccatcagccgcgataacgccaagcgcatggtgtatctgcagatgaacagtctgcgcgccgaggacaccgccgtgtattattgtgccgccggcagcgccagcggctggagcacctatagcccacgccgcctgtatcgctacaattactggggccaaggcacccaagtgaccgtgagcagc

SEQ ID NO: 30 - protein, 128 aa, synthetic construct
  REGION 1..128: note = 505B12 VHH amino acid sequence
EVQLVESGGGLVQPGGSLRLSCAASGFIFSRYIMGWFRQAPGKGRELVAGINAGGGSTYYPDSVEGRFTISRDNAKRMVYLQMNSLRAEDTAVYYCAAGSASGWSTYSPRRLYRYNYWGQGTQVTVSS

SEQ ID NO: 31 - DNA, 363 bp, synthetic construct
  misc_feature 1..363: note = 505D2 VHH nucleotide sequence
  source 1..363: mol_type = other DNA
gaggtgcagctggtggagagcggtggtggtctcgtgcagcccggcggtagtctgcgcctcagctgtgccgccagcggttatatctttagccgctatgccatgggctggtttcgccaagcccccggcaaaggtcgcgaactggtggccgccattaaccgcggcggtagcaccacctattacccagatagcgtggaaggccgcttcaccatcagccgcgataacgccaagcgcatggtgtatctgcagatgaacagtctgcgcgccgaggacaccgccgtgtattattgtgccgccggccgctttggcctgggcagccgcacctacgattactggggccaaggcacccaagtgaccgtgagcagc

SEQ ID NO: 32 - protein, 121 aa, synthetic construct
  REGION 1..121: note = 505D2 VHH amino acid sequence
EVQLVESGGGLVQPGGSLRLSCAASGYIFSRYAMGWFRQAPGKGRELVAAINRGGSTTYYPDSVEGRFTISRDNAKRMVYLQMNSLRAEDTAVYYCAAGRFGLGSRTYDYWGQGTQVTVSS

SEQ ID NO: 33 - DNA, 372 bp, synthetic construct
  misc_feature 1..372: note = 505F1 VHH nucleotide sequence
  source 1..372: mol_type = other DNA
gaggtgcagctggtggagagcggtggtggtctcgtgcagcccggcggtagtctgcgcctcagctgtgccgccagcggtcgcacccttagcaacaataccatgggctggtttcgccaagcccccggcaaaggtcgcgaactggtggccagcattagcgccagcggtagccgcacccactacccagatagcgtggaaggccgcttcaccatcagccgcgataacgccaagcgcatggtgtatctgcagatgaacagtctgcgcgccgaggacaccgccgtgtattattgtgccgccgtgagccgcgtgggcttttatacccgcggcgccacctacaattactggggccaaggcacccaagtgaccgtgagcagc

SEQ ID NO: 34 - protein, 124 aa, synthetic construct
  REGION 1..124: note = 505F1 VHH amino acid sequence
EVQLVESGGGLVQPGGSLRLSCAASGRTLSNNTMGWFRQAPGKGRELVASISASGSRTHYPDSVEGRFTISRDNAKRMVYLQMNSLRAEDTAVYYCAAVSRVGFYTRGATYNYWGQGTQVTVSS

SEQ ID NO: 35 - DNA, 363 bp, synthetic construct
  misc_feature 1..363: note = 505H3 VHH nucleotide sequence
  source 1..363: mol_type = other DNA
gaggtgcagctggtggagagcggtggtggtctcgtgcagcccggcggtagtctgcgcctcagctgtgccgccagcggtaacatccttagcatcaatatcatgggctggtttcgccaagcccccggcaaaggtcgcgaactggtggccgccatttcccgcacgggcggtagcacctactacccagatagcgtggaaggccgcttcaccatcagccgcgataacgccaagcgcatggtgtatctgcagatgaacagtctgcgcgccgaggacaccgccgtgtattattgtgccgccagcagccgccgcagcagcctgaacacctacaattactggggccaaggcacccaagtgaccgtgagcagc

SEQ ID NO: 36 - protein, 121 aa, synthetic construct
  REGION 1..121: note = 505H3 VHH amino acid sequence
EVQLVESGGGLVQPGGSLRLSCAASGNILSINIMGWFRQAPGKGRELVAAISRTGGSTYYPDSVEGRFTISRDNAKRMVYLQMNSLRAEDTAVYYCAASSRRSSLNTYNYWGQGTQVTVSS

SEQ ID NO: 37 - DNA, 363 bp, synthetic construct
  misc_feature 1..363: note = 505H8 VHH nucleotide sequence
  source 1..363: mol_type = other DNA
gaggtgcagctggtggagagcggtggtggtctcgtgcagcccggcggtagtctgcgcctcagctgtgccgccagcggttttatctttagccgcaatgccatgggctggtttcgccaagcccccggcaaaggtcgcgaactggtggccgccattacctggagcggtggcaccacctattacccagatagcgtggaaggccgcttcaccatcagccgcgataacgccaagcgcatggtgtatctgcagatgaacagtctgcgcgccgaggacaccgccgtgtattattgtgccgcccgcatcgcctatagcagcacctggacctacgattactggggccaaggcacccaagtgaccgtgagcagc

SEQ ID NO: 38 - protein, 121 aa, synthetic construct
  REGION 1..121: note = 505H8 VHH amino acid sequence
EVQLVESGGGLVQPGGSLRLSCAASGFIFSRNAMGWFRQAPGKGRELVAAITWSGGTTYYPDSVEGRFTISRDNAKRMVYLQMNSLRAEDTAVYYCAARIAYSSTWTYDYWGQGTQVTVSS

SEQ ID NO: 39 - DNA, 363 bp, synthetic construct
  misc_feature 1..363: note = 505H10 VHH nucleotide sequence
  source 1..363: mol_type = other DNA
gaggtgcagctggtggagagcggtggtggtctcgtgcagcccggcggtagtctgcgcctcagctgtgccgccagcggttttatctttagccgctattatatgggctggtttcgccaagcccccggcaaaggtcgcgaactggtggccgccatttcccgcacgggcggtagcacctactacccagatagcgtggaaggccgcttcaccatcagccgcgataacgccaagcgcatggtgtatctgcagatgaacagtctgcgcgccgaggacaccgccgtgtattattgtgccgccgatctgtatccaggctttcgccgcggctacaattactggggccaaggcacccaagtgaccgtgagcagc

SEQ ID NO: 40 - protein, 121 aa, synthetic construct
  REGION 1..121: note = 505H10 VHH amino acid sequence
EVQLVESGGGLVQPGGSLRLSCAASGFIFSRYYMGWFRQAPGKGRELVAAISRTGGSTYYPDSVEGRFTISRDNAKRMVYLQMNSLRAEDTAVYYCAADLYPGFRRGYNYWGQGTQVTVSS

SEQ ID NO: 41 - DNA, 372 bp, synthetic construct
  misc_feature 1..372: note = 506A5 VHH nucleotide sequence
  source 1..372: mol_type = other DNA
gaggtgcagctggtggagagcggtggtggtctcgtgcagcccggcggtagtctgcgcctcagctgtgccgccagcggttttatctttagccgctatgccatgggctggtttcgccaagcccccggcaaaggtcgcgaactggtggccgccattagccgcggcgatagcgatacctattacccagatagcgtggaaggccgcttcaccatcagccgcgataacgccaagcgcatggtgtatctgcagatgaacagtctgcgcgccgaggacaccgccgtgtattattgtgccgccgtgggccgctattattatggctattatgccaacaactacaattactggggccaaggcacccaagtgaccgtgagcagc

SEQ ID NO: 42 - protein, 124 aa, synthetic construct
  REGION 1..124: note = 506A5 VHH amino acid sequence
EVQLVESGGGLVQPGGSLRLSCAASGFIFSRYAMGWFRQAPGKGRELVAAISRGDSDTYYPDSVEGRFTISRDNAKRMVYLQMNSLRAEDTAVYYCAAVGRYYYGYYANNYNYWGQGTQVTVSS

SEQ ID NO: 43 - DNA, 363 bp, synthetic construct
  misc_feature 1..363: note = 506A8 VHH nucleotide sequence
  source 1..363: mol_type = other DNA
gaggtgcagctggtggagagcggtggtggtctcgtgcagcccggcggtagtctgcgcctcagctgtgccgccagcggttttatctttagccgctatgccatgggctggtttcgccaagcccccggcaaaggtcgcgaactggtggccgccattaaccgcggcgatagcgtgacctattacccagatagcgtggaaggccgcttcaccatcagccgcgataacgccaagcgcatggtgtatctgcagatgaacagtctgcgcgccgaggacaccgccgtgtattattgtgccgcccgcggccgcaccagcctggcctatacctacgattactggggccaaggcacccaagtgaccgtgagcagc

SEQ ID NO: 44 - protein, 121 aa, synthetic construct
  REGION 1..121: note = 506A8 VHH amino acid sequence
EVQLVESGGGLVQPGGSLRLSCAASGFIFSRYAMGWFRQAPGKGRELVAAINRGDSVTYYPDSVEGRFTISRDNAKRMVYLQMNSLRAEDTAVYYCAARGRTSLAYTYDYWGQGTQVTVSS

SEQ ID NO: 45 - DNA, 372 bp, synthetic construct
  misc_feature 1..372: note = 506B6 VHH nucleotide sequence
  source 1..372: mol_type = other DNA
gaggtgcagctggtggagagcggtggtggtctcgtgcagcccggcggtagtctgcgcctcagctgtgccgccagcggttttatctttagccgctatgccatgggctggtttcgccaagcccccggcaaaggtcgcgaactggtggccgccattaacgccggcggtggcaccaccaactacccagatagcgtggaaggccgcttcaccatcagccgcgataacgccaagcgcatggtgtatctgcagatgaacagtctgcgcgccgaggacaccgccgtgtattattgtgccgcctttaccaaacgcagcctgctgaccggcagcgccgtgtacaattactggggccaaggcacccaagtgaccgtgagcagc

SEQ ID NO: 46 - protein, 124 aa, synthetic construct
  REGION 1..124: note = 506B6 VHH amino acid sequence
EVQLVESGGGLVQPGGSLRLSCAASGFIFSRYAMGWFRQAPGKGRELVAAINAGGGTTNYPDSVEGRFTISRDNAKRMVYLQMNSLRAEDTAVYYCAAFTKRSLLTGSAVYNYWGQGTQVTVSS

SEQ ID NO: 47 - DNA, 363 bp, synthetic construct
  misc_feature 1..363: note = 506B12 VHH nucleotide sequence
  source 1..363: mol_type = other DNA
gaggtgcagctggtggagagcggtggtggtctcgtgcagcccggcggtagtctgcgcctcagctgtgccgccagcggtctgatctttagccgcaatgccatgggctggtttcgccaagcccccggcaaaggtcgcgaactggtggccgccattaactggggcggtggcaccacctattacccagatagcgtggaaggccgcttcaccatcagccgcgataacgccaagcgcatggtgtatctgcagatgaacagtctgcgcgccgaggacaccgccgtgtattattgtgccgccaccacccgcaccagccgcccatatacctacaattactggggccaaggcacccaagtgaccgtgagcagc

SEQ ID NO: 48 - protein, 121 aa, synthetic construct
  REGION 1..121: note = 506B12 VHH amino acid sequence
EVQLVESGGGLVQPGGSLRLSCAASGLIFSRNAMGWFRQAPGKGRELVAAINWGGGTTYYPDSVEGRFTISRDNAKRMVYLQMNSLRAEDTAVYYCAATTRTSRPYTYNYWGQGTQVTVSS

SEQ ID NO: 49 - DNA, 384 bp, synthetic construct
  misc_feature 1..384: note = 506C2 VHH nucleotide sequence
  source 1..384: mol_type = other DNA
gaggtgcagctggtggagagcggtggtggtctcgtgcagcccggcggtagtctgcgcctcagctgtgccgccagcggttatatctttagcaacgatgtgatgggctggtttcgccaagcccccggcaaaggtcgcgaactggtggccgccatttcccgcacgggcggtagcacctactacccagatagcgtggaaggccgcttcaccatcagccgcgataacgccaagcgcatggtgtatctgcagatgaacagtctgcgcgccgaggacaccgccgtgtattattgtgccgccagcacccgccgccgctatgccaccgtggattatcgccgcgattatacctacgattactggggccaaggcacccaagtgaccgtgagcagc

SEQ ID NO: 50 - protein, 128 aa, synthetic construct
  REGION 1..128: note = 506C2 VHH amino acid sequence
EVQLVESGGGLVQPGGSLRLSCAASGYIFSNDVMGWFRQAPGKGRELVAAISRTGGSTYYPDSVEGRFTISRDNAKRMVYLQMNSLRAEDTAVYYCAASTRRRYATVDYRRDYTYDYWGQGTQVTVSS

SEQ ID NO: 51 - DNA, 363 bp, synthetic construct
  misc_feature 1..363: note = 506C5 VHH nucleotide sequence
  source 1..363: mol_type = other DNA
gaggtgcagctggtggagagcggtggtggtctcgtgcagcccggcggtagtctgcgcctcagctgtgccgccagcggttttatctttagccgctattatatgggctggtttcgccaagcccccggcaaaggtcgcgaactggtggcccgcattaccagcggcgatggcagcacctattacccagatagcgtggaaggccgcttcaccatcagccgcgataacgccaagcgcatggtgtatctgcagatgaacagtctgcgcgccgaggacaccgccgtgtattattgtgccgcccgcagctttcgccgcgatatctatgattacaattactggggccaaggcacccaagtgaccgtgagcagc

SEQ ID NO: 52 - protein, 121 aa, synthetic construct
  REGION 1..121: note = 506C5 VHH amino acid sequence
EVQLVESGGGLVQPGGSLRLSCAASGFIFSRYYMGWFRQAPGKGRELVARITSGDGSTYYPDSVEGRFTISRDNAKRMVYLQMNSLRAEDTAVYYCAARSFRRDIYDYNYWGQGTQVTVSS

SEQ ID NO: 53 - DNA, 363 bp, synthetic construct
  misc_feature 1..363: note = 506C8 VHH nucleotide sequence
  source 1..363: mol_type = other DNA
gaggtgcagctggtggagagcggtggtggtctcgtgcagcccggcggtagtctgcgcctcagctgtgccgccagcggttatatctttagcaactatgccatgggctggtttcgccaagcccccggcaaaggtcgcgaactggtggccagcattaaccgcagcggtagcatcacctattacccagatagcgtggaaggccgcttcaccatcagccgcgataacgccaagcgcatggtgtatctgcagatgaacagtctgcgcgccgaggacaccgccgtgtattattgtgccgccaacgatgtgcgcggctattatcgccgctacaattactggggccaaggcacccaagtgaccgtgagcagc

SEQ ID NO: 54 - protein, 121 aa, synthetic construct
  REGION 1..121: note = 506C8 VHH amino acid sequence
EVQLVESGGGLVQPGGSLRLSCAASGYIFSNYAMGWFRQAPGKGRELVASINRSGSITYYPDSVEGRFTISRDNAKRMVYLQMNSLRAEDTAVYYCAANDVRGYYRRYNYWGQGTQVTVSS

SEQ ID NO: 55 - DNA, 363 bp, synthetic construct
  misc_feature 1..363: note = 506C11 VHH nucleotide sequence
  source 1..363: mol_type = other DNA
gaggtgcagctggtggagagcggtggtggtctcgtgcagcccggcggtagtctgcgcctcagctgtgccgccagcggtctgatctttagcagctatgccatgggctggtttcgccaagcccccggcaaaggtcgcgaactggtggccagcattaaccgccgcggtggcagcacctattacccagatagcgtggaaggccgcttcaccatcagccgcgataacgccaagcgcatggtgtatctgcagatgaacagtctgcgcgccgaggacaccgccgtgtattattgtgccgccggcagccgcagcagcagccgcctgggctacaattactggggccaaggcacccaagtgaccgtgagcagc

SEQ ID NO: 56 - protein, 121 aa, synthetic construct
  REGION 1..121: note = 506C11 VHH amino acid sequence
EVQLVESGGGLVQPGGSLRLSCAASGLIFSSYAMGWFRQAPGKGRELVASINRRGGSTYYPDSVEGRFTISRDNAKRMVYLQMNSLRAEDTAVYYCAAGSRSSSRLGYNYWGQGTQVTVSS

SEQ ID NO: 57 - DNA, 363 bp, synthetic construct
  misc_feature 1..363: note = 506D2 VHH nucleotide sequence
  source 1..363: mol_type = other DNA
gaggtgcagctggtggagagcggtggtggtctcgtgcagcccggcggtagtctgcgcctcagctgtgccgccagcggtatcatctttagccgctatgccatgggctggtttcgccaagcccccggcaaaggtcgcgaactggtggccgccattaaccgcagcggtggccgcaccagctacccagatagcgtggaaggccgcttcaccatcagccgcgataacgccaagcgcatggtgtatctgcagatgaacagtctgcgcgccgaggacaccgccgtgtattattgtgccgcctttctggccagctgggatggcaccacctacgattactggggccaaggcacccaagtgaccgtgagcagc

SEQ ID NO: 58 - protein, 121 aa, synthetic construct
  REGION 1..121: note = 506D2 VHH amino acid sequence
EVQLVESGGGLVQPGGSLRLSCAASGIIFSRYAMGWFRQAPGKGRELVAAINRSGGRTSYPDSVEGRFTISRDNAKRMVYLQMNSLRAEDTAVYYCAAFLASWDGTTYDYWGQGTQVTVSS

SEQ ID NO: 59 - DNA, 384 bp, synthetic construct
  misc_feature 1..384: note = 506D8 VHH nucleotide sequence
  source 1..384: mol_type = other DNA
gaggtgcagctggtggagagcggtggtggtctcgtgcagcccggcggtagtctgcgcctcagctgtgccgccagcggttatacccttagcagctattatatgggctggtttcgccaagcccccggcaaaggtcgcgaactggtggccgccattacctggggcggtggcagcacctattacccagatagcgtggaaggccgcttcaccatcagccgcgataacgccaagcgcatggtgtatctgcagatgaacagtctgcgcgccgaggacaccgccgtgtattattgtgccgccgcccgcaaacgcagcgtgacctataccaccctgagctatgcctatagctacgattactggggccaaggcacccaagtgaccgtgagcagc

SEQ ID NO: 60 - protein, 128 aa, synthetic construct
  REGION 1..128: note = 506D8 VHH amino acid sequence
EVQLVESGGGLVQPGGSLRLSCAASGYTLSSYYMGWFRQAPGKGRELVAAITWGGGSTYYPDSVEGRFTISRDNAKRMVYLQMNSLRAEDTAVYYCAAARKRSVTYTTLSYAYSYDYWGQGTQVTVSS

SEQ ID NO: 61 - DNA, 357 bp, synthetic construct
  misc_feature 1..357: note = 506E1 VHH nucleotide sequence
  source 1..357: mol_type = other DNA
gaggtgcagctggtggagagcggtggtggtctcgtgcagcccggcggtagtctgcgcctcagctgtgccgccagcggttatatctttagccgctatagcatgggctggtttcgccaagcccccggcaaaggtcgcgaactggtggccgccattagcagcagcggtagcagcacctattacccagatagcgtggaaggccgcttcaccatcagccgcgataacgccaagcgcatggtgtatctgcagatgaacagtctgcgcgccgaggacaccgccgtgtattattgtgccgccaccccacgccgcagcaccggcaacaccttttggggccaaggcacccaagtgaccgtgagcagc

SEQ ID NO: 62 - protein, 119 aa, synthetic construct
  REGION 1..119: note = 506E1 VHH amino acid sequence
EVQLVESGGGLVQPGGSLRLSCAASGYIFSRYSMGWFRQAPGKGRELVAAISSSGSSTYYPDSVEGRFTISRDNAKRMVYLQMNSLRAEDTAVYYCAATPRRSTGNTFWGQGTQVTVSS

SEQ ID NO: 63 - DNA, 372 bp, synthetic construct
  misc_feature 1..372: note = 506F5 VHH nucleotide sequence
  source 1..372: mol_type = other DNA
gaggtgcagctggtggagagcggtggtggtctcgtgcagcccggcggtagtctgcgcctcagctgtgccgccagcggtggcatctttagcagctatgccatgggctggtttcgccaagcccccggcaaaggtcgcgaactggtggccgccattaaccgcggcggtggcggcacctattacccagatagcgtggaaggccgcttcaccatcagccgcgataacgccaagcgcatggtgtatctgcagatgaacagtctgcgcgccgaggacaccgccgtgtattattgtgccgcctttggccgctatagccgcggcagcgatgatagccgctacaattactggggccaaggcacccaagtgaccgtgagcagc

SEQ ID NO: 64 - protein, 124 aa, synthetic construct
  REGION 1..124: note = 506F5 VHH amino acid sequence
EVQLVESGGGLVQPGGSLRLSCAASGGIFSSYAMGWFRQAPGKGRELVAAINRGGGGTYYPDSVEGRFTISRDNAKRMVYLQMNSLRAEDTAVYYCAAFGRYSRGSDDSRYNYWGQGTQVTVSS

SEQ ID NO: 65 - DNA, 363 bp, synthetic construct
  misc_feature 1..363: note = 506G1 VHH nucleotide sequence
  source 1..363: mol_type = other DNA
gaggtgcagctggtggagagcggtggtggtctcgtgcagcccggcggtagtctgcgcctcagctgtgccgccagcggttttatctttagccgctatgccatgggctggtttcgccaagcccccggcaaaggtcgcgaactggtggccgccattagctggagcggtggcagcacctattacccagatagcgtggaaggccgcttcaccatcagccgcgataacgccaagcgcatggtgtatctgcagatgaacagtctgcgcgccgaggacaccgccgtgtattattgtgccgccggcagccgcagcagcagccgcctgggctacaattactggggccaaggcacccaagtgaccgtgagcagc

SEQ ID NO: 66 - protein, 121 aa, synthetic construct
  REGION 1..121: note = 506G1 VHH amino acid sequence
EVQLVESGGGLVQPGGSLRLSCAASGFIFSRYAMGWFRQAPGKGRELVAAISWSGGSTYYPDSVEGRFTISRDNAKRMVYLQMNSLRAEDTAVYYCAAGSRSSSRLGYNYWGQGTQVTVSS

SEQ ID NO: 67 - DNA, 360 bp, synthetic construct
  misc_feature 1..360: note = 506H2 VHH nucleotide sequence
  source 1..360: mol_type = other DNA
gaggtgcagctggtggagagcggtggtggtctcgtgcagcccggcggtagtctgcgcctcagctgtgccgccagcggtcgcacctttagctattataccatgggctggtttcgccaagcccccggcaaaggtcgcgaactggtggccgctaccagccgcgatggcagcacctattacccagatagcgtggaaggccgcttcaccatcagccgcgataacgccaagcgcatggtgtatctgcagatgaacagtctgcgcgccgaggacaccgccgtgtattattgtgccgccgtgcgccgctggagcagcgatagcacctacaattactggggccaaggcacccaagtgaccgtgagcagc

SEQ ID NO: 68 - protein, 120 aa, synthetic construct
  REGION 1..120: note = 506H2 VHH amino acid sequence
EVQLVESGGGLVQPGGSLRLSCAASGRTFSYYTMGWFRQAPGKGRELVAATSRDGSTYYPDSVEGRFTISRDNAKRMVYLQMNSLRAEDTAVYYCAAVRRWSSDSTYNYWGQGTQVTVSS

SEQ ID NO: 69 - DNA, 372 bp, synthetic construct
  misc_feature 1..372: note = 506H9 VHH nucleotide sequence
  source 1..372: mol_type = other DNA
gaggtgcagctggtggagagcggtggtggtctcgtgcagcccggcggtagtctgcgcctcagctgtgccgccagcggtcgcacctttagccgctatgccatgggctggtttcgccaagcccccggcaaaggtcgcgaactggtggccgccattagcagccgcggtagcaccaccaactacccagatagcgtggaaggccgcttcaccatcagccgcgataacgccaagcgcatggtgtatctgcagatgaacagtctgcgcgccgaggacaccgccgtgtattattgtgccgccagcctgtatgtgatcccagcctggaacgaatatggctacaattactggggccaaggcacccaagtgaccgtgagcagc

SEQ ID NO: 70 - protein, 124 aa, synthetic construct
  REGION 1..124: note = 506H9 VHH amino acid sequence
EVQLVESGGGLVQPGGSLRLSCAASGRTFSRYAMGWFRQAPGKGRELVAAISSRGSTTNYPDSVEGRFTISRDNAKRMVYLQMNSLRAEDTAVYYCAASLYVIPAWNEYGYNYWGQGTQVTVSS

SEQ ID NO: 71 - DNA, 63 bp, synthetic construct
  misc_feature 1..63: note = nucleotide sequence of CD8 signal peptide
  source 1..63: mol_type = other DNA
atggctctgcctgtgaccgctctgctgctgcctctggctctgctgctgcacgccgcaagacct

SEQ ID NO: 72 - protein, 21 aa, synthetic construct
  REGION 1..21: note = amino acid sequence of CD8 signal peptide
MALPVTALLLPLALLLHAARP

SEQ ID NO: 73 - DNA, 135 bp, synthetic construct
  misc_feature 1..135: note = nucleotide sequence of CD8 hinge region
  source 1..135: mol_type = other DNA
accacgacgccagcgccgcgaccaccaacaccggcgcccaccatcgcgtcgcagcccctgtccctgcgcccagaggcgtgccggccagcggcggggggcgcagtgcacacgagggggctggacttcgcctgtgat

SEQ ID NO: 74 - protein, 45 aa, synthetic construct
  REGION 1..45: note = amino acid sequence of CD8 hinge region
TTTPAPRPPTPAPTIASQPLSLRPEACRPAAGGAVHTRGLDFACD

SEQ ID NO: 75 - DNA, 72 bp, synthetic construct
  misc_feature 1..72: note = nucleotide sequence of CD8 transmembrane region
  source 1..72: mol_type = other DNA
atctacatctgggcgcccttggccgggacttgtggggtccttctcctgtcactggttatcaccctttactgc

SEQ ID NO: 76 - protein, 24 aa, synthetic construct
  REGION 1..24: note = amino acid sequence of CD8 transmembrane region
IYIWAPLAGTCGVLLLSLVITLYC

SEQ ID NO: 77 - DNA, 126 bp, synthetic construct
  misc_feature 1..126: note = CD137(4-1BB) nucleotide sequence
  source 1..126: mol_type = other DNA
aaacggggcagaaagaaactcctgtatatattcaaacaaccatttatgagaccagtacaaactactcaagaggaagatggctgtagctgccgatttccagaagaagaagaaggaggatgtgaactg

SEQ ID NO: 78 - protein, 42 aa, synthetic construct
  REGION 1..42: note = CD137(4-1BB) amino acid sequence
KRGRKKLLYIFKQPFMRPVQTTQEEDGCSCRFPEEEEGGCEL

SEQ ID NO: 79 - DNA, 336 bp, synthetic construct
  misc_feature 1..336: note = CD3zeta nucleotide sequence
  source 1..336: mol_type = other DNA
agagtgaagttcagcaggagcgcagacgcccccgcgtaccagcagggccagaaccagctctataacgagctcaatctaggacgaagagaggagtacgatgttttggacaagagacgtggccgggaccctgagatggggggaaagccgagaaggaagaaccctcaggaaggcctgtacaatgaactgcagaaagataagatggcggaggcctacagtgagattgggatgaaaggcgagcgccggaggggcaaggggcacgatggcctttaccagggtctcagtacagccaccaaggacacctacgacgcccttcacatgcaggccctgccccctcgc

SEQ ID NO: 80 - protein, 112 aa, synthetic construct
  REGION 1..112: note = CD3zeta amino acid sequence
RVKFSRSADAPAYQQGQNQLYNELNLGRREEYDVLDKRRGRDPEMGGKPRRKNPQEGLYNELQKDKMAEAYSEIGMKGERRRGKGHDGLYQGLSTATKDTYDALHMQALPPR

SEQ ID NO: 81 - DNA, 54 bp, synthetic construct
  misc_feature 1..54: note = T2A nucleotide sequence
  source 1..54: mol_type = other DNA
gagggcagaggaagtcttctaacatgcggtgacgtggaggagaatcccggccct

SEQ ID NO: 82 - protein, 18 aa, synthetic construct
  REGION 1..18: note = T2A amino acid sequence
EGRGSLLTCGDVEENPGP

SEQ ID NO: 83 - DNA, 1194 bp, synthetic construct
  misc_feature 1..1194: note = Ori2 nucleotide sequence
  source 1..1194: mol_type = other DNA
atgggggccgtcctgaggagcctcctggcctgcagcttctgtgtgctcctgagagcggagcagaaactcatctctgaagaggatctggaacctccaacatgttctcctcagcagtttacttgtttcacgggggaaattgactgtatccctgtggcttggcggtgcgatgggtttactgaatgtgaagaccacagtgatgaactcaattgtcctgtatgctcagagtcccagttccagtgtgccagtgggcagtgtattgatggtgccctccgatgcaatggagatgcaaactgccaggacaaatcagatgagaagaactgtgaagtgctttgtttaattgatcagttccgctgtgccaatggtcagtgcattggaaagcacaagaagtgtgatcataatgtggattgcagtgacaagtcagatgaactggattgttatccgactgaagaaccagcaccacaggccaccaatacagttggttctgttattggcgtaattgtcaccatttttgtgtctggaactgtatactttatctgccagaggatgttgtgtccacgtatgaagggagatggggaaactatgactaatgactatgtagttcatggaccagcttctgtgcctcttggttatgtgccacacccaagttctttgtcaggatctcttccaggaatgtctcgaggtaaatcaatgatcagctccctcagtatcatggggggaagcagtggacccccctatgaccgagcccatgttacaggagcatcatcaagtagttcttcaagcaccaaaggcacttacttccctgcaattttgaaccctccaccatccccagccacagagcgatcacattacactatggaatttggatattcttcaaacagtccttccactcataggtcatacagctacaggccatatagctaccggcactttgcaccccccaccacaccctgcagcacagatgtttgtgacagtgactatgctcctagtcggagaatgacctcagtggcaacagccaagggctataccagtgacttgaactatgattcagaacctgtgcccccacctcccacaccccgaagccaatacttgtcagcagaggagaactatgaaagctgcccaccttctccatacacagagaggagctattctcatcacctctacccaccgccaccctctccctgtacagactcctcc

SEQ ID NO: 84 - protein, 398 aa, synthetic construct
  REGION 1..398: note = Ori2 amino acid sequence
MGAVLRSLLACSFCVLLRAEQKLISEEDLEPPTCSPQQFTCFTGEIDCIPVAWRCDGFTECEDHSDELNCPVCSESQFQCASGQCIDGALRCNGDANCQDKSDEKNCEVLCLIDQFRCANGQCIGKHKKCDHNVDCSDKSDELDCYPTEEPAPQATNTVGSVIGVIVTIFVSGTVYFICQRMLCPRMKGDGETMTNDYVVHGPASVPLGYVPHPSSLSGSLPGMSRGKSMISSLSIMGGSSGPPYDRAHVTGASSSSSSSTKGTYFPAILNPPPSPATERSHYTMEFGYSSNSPSTHRSYSYRPYSYRHFAPPTTPCSTDVCDSDYAPSRRMTSVATAKGYTSDLNYDSEPVPPPPTPRSQYLSAEENYESCPPSPYTERSYSHHLYPPPPSPCTDSS

SEQ ID NO: 85 - DNA, 2346 bp, synthetic construct
  misc_feature 1..2346: note = 3B5 VHH-ori2 CAR nucleotide sequence
  source 1..2346: mol_type = other DNA
atggctctgcctgtgaccgctctgctgctgcctctggctctgctgctgcacgccgcaagacctgaggtgcagctggtggagagcggtggtggtctcgtgcagcccggcggtagtctgcgcctcagctgtgccgccagcggttttatctttagccgctatggcatgggctggtttcgccaagcccccggcaaaggtcgcgaactggtggccgccattaactggagcgatggcaccacctattacccagatagcgtggaaggccgcttcaccatcagccgcgataacgccaagcgcatggtgtatctgcagatgaacagtctgcgcgccgaggacaccgccgtgtattattgtgccgccgatcgccgcctgcgcagccagaccggctacgattactggggccaaggcacccaagtgaccgtgagcagcaccacgacgccagcgccgcgaccaccaacaccggcgcccaccatcgcgtcgcagcccctgtccctgcgcccagaggcgtgccggccagcggcggggggcgcagtgcacacgagggggctggacttcgcctgtgatatctacatctgggcgcccttggccgggacttgtggggtccttctcctgtcactggttatcaccctttactgcaaacggggcagaaagaaactcctgtatatattcaaacaaccatttatgagaccagtacaaactactcaagaggaagatggctgtagctgccgatttccagaagaagaagaaggaggatgtgaactgagagtgaagttcagcaggagcgcagacgcccccgcgtaccagcagggccagaaccagctctataacgagctcaatctaggacgaagagaggagtacgatgttttggacaagagacgtggccgggaccctgagatggggggaaagccgagaaggaagaaccctcaggaaggcctgtacaatgaactgcagaaagataagatggcggaggcctacagtgagattgggatgaaaggcgagcgccggaggggcaaggggcacgatggcctttaccagggtctcagtacagccaccaaggacacctacgacgcccttcacatgcaggccctgccccctcgcgagggcagaggaagtcttctaacatgcggtgacgtggaggagaatcccggccctatgggggccgtcctgaggagcctcctggcctgcagcttctgtgtgctcctgagagcggagcagaaactcatctctgaagaggatctggaacctccaacatgttctcctcagcagtttacttgtttcacgggggaaattgactgtatccctgtggcttggcggtgcgatgggtttactgaatgtgaagaccacagtgatgaactcaattgtcctgtatgctcagagtcccagttccagtgtgccagtgggcagtgtattgatggtgccctccgatgcaatggagatgcaaactgccaggacaaatcagatgagaagaactgtgaagtgctttgtttaattgatcagttccgctgtgccaatggtcagtgcattggaaagcacaagaagtgtgatcataatgtggattgcagtgacaagtcagatgaactggattgttatccgactgaagaaccagcaccacaggccaccaatacagttggttctgttattggcgtaattgtcaccatttttgtgtctggaactgtatactttatctgccagaggatgttgtgtccacgtatgaagggagatggggaaactatgactaatgactatgtagttcatggaccagcttctgtgcctcttggttatgtgccacacccaagttctttgtcaggatctcttccaggaatgtctcgaggtaaatcaatgatcagctccctcagtatcatggggggaagcagtggacccccctatgaccgagcccatgttacaggagcatcatcaagtagttcttcaagcaccaaaggcacttacttccctgcaattttgaaccctccaccatccccagccacagagcgatcacattacactatggaatttggatattcttcaaacagtccttccactcataggtcatacagctacaggccatatagctaccggcactttgcaccccccaccacaccctgcagcacagatgtttgtgacagtgactatgctcctagtcggagaatgacctcagtggcaacagccaagggctataccagtgacttgaactatgattcagaacctgtgcccccacctcccacaccccgaagccaatacttgtcagcagaggagaactatgaaagctgcccaccttctccatacacagagaggagctattctcatcacctctacccaccgccaccctctccctgtacagactcctcctga

SEQ ID NO: 86 - protein, 782 aa, synthetic construct
  REGION 1..782: note = 3B5 VHH-ori2 CAR amino acid sequence
  SITE 782: note = misc_feature - Xaa = any one kind of amino acid
MALPVTALLLPLALLLHAARPEVQLVESGGGLVQPGGSLRLSCAASGFIFSRYGMGWFRQAPGKGRELVAAINWSDGTTYYPDSVEGRFTISRDNAKRMVYLQMNSLRAEDTAVYYCAADRRLRSQTGYDYWGQGTQVTVSSTTTPAPRPPTPAPTIASQPLSLRPEACRPAAGGAVHTRGLDFACDIYIWAPLAGTCGVLLLSLVITLYCKRGRKKLLYIFKQPFMRPVQTTQEEDGCSCRFPEEEEGGCELRVKFSRSADAPAYQQGQNQLYNELNLGRREEYDVLDKRRGRDPEMGGKPRRKNPQEGLYNELQKDKMAEAYSEIGMKGERRRGKGHDGLYQGLSTATKDTYDALHMQALPPREGRGSLLTCGDVEENPGPMGAVLRSLLACSFCVLLRAEQKLISEEDLEPPTCSPQQFTCFTGEIDCIPVAWRCDGFTECEDHSDELNCPVCSESQFQCASGQCIDGALRCNGDANCQDKSDEKNCEVLCLIDQFRCANGQCIGKHKKCDHNVDCSDKSDELDCYPTEEPAPQATNTVGSVIGVIVTIFVSGTVYFICQRMLCPRMKGDGETMTNDYVVHGPASVPLGYVPHPSSLSGSLPGMSRGKSMISSLSIMGGSSGPPYDRAHVTGASSSSSSSTKGTYFPAILNPPPSPATERSHYTMEFGYSSNSPSTHRSYSYRPYSYRHFAPPTTPCSTDVCDSDYAPSRRMTSVATAKGYTSDLNYDSEPVPPPPTPRSQYLSAEENYESCPPSPYTERSYSHHLYPPPPSPCTDSSX

SEQ ID NO: 87 - DNA, 2355 bp, synthetic construct
  misc_feature 1..2355: note = 3E7 VHH-ori2 CAR nucleotide sequence
  source 1..2355: mol_type = other DNA
atggctctgcctgtgaccgctctgctgctgcctctggctctgctgctgcacgccgcaagacctgaggtgcagctggtggagagcggtggtggtctcgtgcagcccggcggtagtctgcgcctcagctgtgccgccagcggtcgcatctttagccgcgatgccatgggctggtttcgccaagcccccggcaaaggtcgcgaactggtggccgccattaacagcagcggtggcaacacctattacccagatagcgtggaaggccgcttcaccatcagccgcgataacgccaagcgcatggtgtatctgcagatgaacagtctgcgcgccgaggacaccgccgtgtattattgtgccgcccgcggcgtgcgctggaccagcaccaccgcctatggctacaattactggggccaaggcacccaagtgaccgtgagcagcaccacgacgccagcgccgcgaccaccaacaccggcgcccaccatcgcgtcgcagcccctgtccctgcgcccagaggcgtgccggccagcggcggggggcgcagtgcacacgagggggctggacttcgcctgtgatatctacatctgggcgcccttggccgggacttgtggggtccttctcctgtcactggttatcaccctttactgcaaacggggcagaaagaaactcctgtatatattcaaacaaccatttatgagaccagtacaaactactcaagaggaagatggctgtagctgccgatttccagaagaagaagaaggaggatgtgaactgagagtgaagttcagcaggagcgcagacgcccccgcgtaccagcagggccagaaccagctctataacgagctcaatctaggacgaagagaggagtacgatgttttggacaagagacgtggccgggaccctgagatggggggaaagccgagaaggaagaaccctcaggaaggcctgtacaatgaactgcagaaagataagatggcggaggcctacagtgagattgggatgaaaggcgagcgccggaggggcaaggggcacgatggcctttaccagggtctcagtacagccaccaaggacacctacgacgcccttcacatgcaggccctgccccctcgcgagggcagaggaagtcttctaacatgcggtgacgtggaggagaatcccggccctatgggggccgtcctgaggagcctcctggcctgcagcttctgtgtgctcctgagagcggagcagaaactcatctctgaagaggatctggaacctccaacatgttctcctcagcagtttacttgtttcacgggggaaattgactgtatccctgtggcttggcggtgcgatgggtttactgaatgtgaagaccacagtgatgaactcaattgtcctgtatgctcagagtcccagttccagtgtgccagtgggcagtgtattgatggtgccctccgatgcaatggagatgcaaactgccaggacaaatcagatgagaagaactgtgaagtgctttgtttaattgatcagttccgctgtgccaatggtcagtgcattggaaagcacaagaagtgtgatcataatgtggattgcagtgacaagtcagatgaactggattgttatccgactgaagaaccagcaccacaggccaccaatacagttggttctgttattggcgtaattgtcaccatttttgtgtctggaactgtatactttatctgccagaggatgttgtgtccacgtatgaagggagatggggaaactatgactaatgactatgtagttcatggaccagcttctgtgcctcttggttatgtgccacacccaagttctttgtcaggatctcttccaggaatgtctcgaggtaaatcaatgatcagctccctcagtatcatggggggaagcagtggacccccctatgaccgagcccatgttacaggagcatcatcaagtagttcttcaagcaccaaaggcacttacttccctgcaattttgaaccctccaccatccccagccacagagcgatcacattacactatggaatttggatattcttcaaacagtccttccactcataggtcatacagctacaggccatatagctaccggcactttgcaccccccaccacaccctgcagcacagatgtttgtgacagtgactatgctcctagtcggagaatgacctcagtggcaacagccaagggctataccagtgacttgaactatgattcagaacctgtgcccccacctcccacaccccgaagccaatacttgtcagcagaggagaactatgaaagctgcccaccttctccatacacagagaggagctattctcatcacctctacccaccgccaccctctccctgtacagactcctcctga

SEQ ID NO: 88 - protein, 785 aa, synthetic construct
  REGION 1..785: note = 3E7 VHH-ori2 CAR amino acid sequence
  SITE 785: note = misc_feature - Xaa = any one kind of amino acid
MALPVTALLLPLALLLHAARPEVQLVESGGGLVQPGGSLRLSCAASGRIFSRDAMGWFRQAPGKGRELVAAINSSGGNTYYPDSVEGRFTISRDNAKRMVYLQMNSLRAEDTAVYYCAARGVRWTSTTAYGYNYWGQGTQVTVSSTTTPAPRPPTPAPTIASQPLSLRPEACRPAAGGAVHTRGLDFACDIYIWAPLAGTCGVLLLSLVITLYCKRGRKKLLYIFKQPFMRPVQTTQEEDGCSCRFPEEEEGGCELRVKFSRSADAPAYQQGQNQLYNELNLGRREEYDVLDKRRGRDPEMGGKPRRKNPQEGLYNELQKDKMAEAYSEIGMKGERRRGKGHDGLYQGLSTATKDTYDALHMQALPPREGRGSLLTCGDVEENPGPMGAVLRSLLACSFCVLLRAEQKLISEEDLEPPTCSPQQFTCFTGEIDCIPVAWRCDGFTECEDHSDELNCPVCSESQFQCASGQCIDGALRCNGDANCQDKSDEKNCEVLCLIDQFRCANGQCIGKHKKCDHNVDCSDKSDELDCYPTEEPAPQATNTVGSVIGVIVTIFVSGTVYFICQRMLCPRMKGDGETMTNDYVVHGPASVPLGYVPHPSSLSGSLPGMSRGKSMISSLSIMGGSSGPPYDRAHVTGASSSSSSSTKGTYFPAILNPPPSPATERSHYTMEFGYSSNSPSTHRSYSYRPYSYRHFAPPTTPCSTDVCDSDYAPSRRMTSVATAKGYTSDLNYDSEPVPPPPTPRSQYLSAEENYESCPPSPYTERSYSHHLYPPPPSPCTDSSX

SEQ ID NO: 89 - DNA, 2355 bp, synthetic construct
  misc_feature 1..2355: note = 4A2 VHH-ori2 CAR nucleotide sequence
  source 1..2355: mol_type = other DNA
atggctctgcctgtgaccgctctgctgctgcctctggctctgctgctgcacgccgcaagacctgaggtgcagctggtggagagcggtggtggtctcgtgcagcccggcggtagtctgcgcctcagctgtgccgccagcggttttatctttagccgctatgatatgggctggtttcgccaagcccccggcaaaggtcgcgaactggtggccgtgattacctggggcggtggcagcacctattacccagatagcgtggaaggccgcttcaccatcagccgcgataacgccaagcgcatggtgtatctgcagatgaacagtctgcgcgccgaggacaccgccgtgtattattgtgccgcccgcagcgccagcgcctatcgcaccggccgcctggaatacaattactggggccaaggcacccaagtgaccgtgagcagcaccacgacgccagcgccgcgaccaccaacaccggcgcccaccatcgcgtcgcagcccctgtccctgcgcccagaggcgtgccggccagcggcggggggcgcagtgcacacgagggggctggacttcgcctgtgatatctacatctgggcgcccttggccgggacttgtggggtccttctcctgtcactggttatcaccctttactgcaaacggggcagaaagaaactcctgtatatattcaaacaaccatttatgagaccagtacaaactactcaagaggaagatggctgtagctgccgatttccagaagaagaagaaggaggatgtgaactgagagtgaagttcagcaggagcgcagacgcccccgcgtaccagcagggccagaaccagctctataacgagctcaatctaggacgaagagaggagtacgatgttttggacaagagacgtggccgggaccctgagatggggggaaagccgagaaggaagaaccctcaggaaggcctgtacaatgaactgcagaaagataagatggcggaggcctacagtgagattgggatgaaaggcgagcgccggaggggcaaggggcacgatggcctttaccagggtctcagtacagccaccaaggacacctacgacgcccttcacatgcaggccctgccccctcgcgagggcagaggaagtcttctaacatgcggtgacgtggaggagaatcccggccctatgggggccgtcctgaggagcctcctggcctgcagcttctgtgtgctcctgagagcggagcagaaactcatctctgaagaggatctggaacctccaacatgttctcctcagcagtttacttgtttcacgggggaaattgactgtatccctgtggcttggcggtgcgatgggtttactgaatgtgaagaccacagtgatgaactcaattgtcctgtatgctcagagtcccagttccagtgtgccagtgggcagtgtattgatggtgccctccgatgcaatggagatgcaaactgccaggacaaatcagatgagaagaactgtgaagtgctttgtttaattgatcagttccgctgtgccaatggtcagtgcattggaaagcacaagaagtgtgatcataatgtggattgcagtgacaagtcagatgaactggattgttatccgactgaagaaccagcaccacaggccaccaatacagttggttctgttattggcgtaattgtcaccatttttgtgtctggaactgtatactttatctgccagaggatgttgtgtccacgtatgaagggagatggggaaactatgactaatgactatgtagttcatggaccagcttctgtgcctcttggttatgtgccacacccaagttctttgtcaggatctcttccaggaatgtctcgaggtaaatcaatgatcagctccctcagtatcatggggggaagcagtggacccccctatgaccgagcccatgttacaggagcatcatcaagtagttcttcaagcaccaaaggcacttacttccctgcaattttgaaccctccaccatccccagccacagagcgatcacattacactatggaatttggatattcttcaaacagtccttccactcataggtcatacagctacaggccatatagctaccggcactttgcaccccccaccacaccctgcagcacagatgtttgtgacagtgactatgctcctagtcggagaatgacctcagtggcaacagccaagggctataccagtgacttgaactatgattcagaacctgtgcccccacctcccacaccccgaagccaatacttgtcagcagaggagaactatgaaagctgcccaccttctccatacacagagaggagctattctcatcacctctacccaccgccaccctctccctgtacagactcctcctga

SEQ ID NO: 90 - protein, 785 aa, synthetic construct
  REGION 1..785: note = 4A2 VHH-ori2 CAR amino acid sequence
  SITE 785: note = misc_feature - Xaa = any one kind of amino acid
MALPVTALLLPLALLLHAARPEVQLVESGGGLVQPGGSLRLSCAASGFIFSRYDMGWFRQAPGKGRELVAVITWGGGSTYYPDSVEGRFTISRDNAKRMVYLQMNSLRAEDTAVYYCAARSASAYRTGRLEYNYWGQGTQVTVSSTTTPAPRPPTPAPTIASQPLSLRPEACRPAAGGAVHTRGLDFACDIYIWAPLAGTCGVLLLSLVITLYCKRGRKKLLYIFKQPFMRPVQTTQEEDGCSCRFPEEEEGGCELRVKFSRSADAPAYQQGQNQLYNELNLGRREEYDVLDKRRGRDPEMGGKPRRKNPQEGLYNELQKDKMAEAYSEIGMKGERRRGKGHDGLYQGLSTATKDTYDALHMQALPPREGRGSLLTCGDVEENPGPMGAVLRSLLACSFCVLLRAEQKLISEEDLEPPTCSPQQFTCFTGEIDCIPVAWRCDGFTECEDHSDELNCPVCSESQFQCASGQCIDGALRCNGDANCQDKSDEKNCEVLCLIDQFRCANGQCIGKHKKCDHNVDCSDKSDELDCYPTEEPAPQATNTVGSVIGVIVTIFVSGTVYFICQRMLCPRMKGDGETMTNDYVVHGPASVPLGYVPHPSSLSGSLPGMSRGKSMISSLSIMGGSSGPPYDRAHVTGASSSSSSSTKGTYFPAILNPPPSPATERSHYTMEFGYSSNSPSTHRSYSYRPYSYRHFAPPTTPCSTDVCDSDYAPSRRMTSVATAKGYTSDLNYDSEPVPPPPTPRSQYLSAEENYESCPPSPYTERSYSHHLYPPPPSPCTDSSX

SEQ ID NO: 91 - DNA, 2346 bp, synthetic construct
  misc_feature 1..2346: note = 4B3 VHH-ori2 CAR nucleotide sequence
  source 1..2346: mol_type = other DNA
atggctctgcctgtgaccgctctgctgctgcctctggctctgctgctgcacgccgcaagacctgaggtgcagctggtggagagcggtggtggtctcgtgcagcccggcggtagtctgcgcctcagctgtgccgccagcggtctgatctttagccgctatgtgatgggctggtttcgccaagcccccggcaaaggtcgcgaactggtggcctttattaacagcagcggtggcagcaccaactacccagatagcgtggaaggccgcttcaccatcagccgcgataacgccaagcgcatggtgtatctgcagatgaacagtctgcgcgccgaggacaccgccgtgtattattgtgccgccagcagccgcaccagcaccacccgcggctacaattactggggccaaggcacccaagtgaccgtgagcagcaccacgacgccagcgccgcgaccaccaacaccggcgcccaccatcgcgtcgcagcccctgtccctgcgcccagaggcgtgccggccagcggcggggggcgcagtgcacacgagggggctggacttcgcctgtgatatctacatctgggcgcccttggccgggacttgtggggtccttctcctgtcactggttatcaccctttactgcaaacggggcagaaagaaactcctgtatatattcaaacaaccatttatgagaccagtacaaactactcaagaggaagatggctgtagctgccgatttccagaagaagaagaaggaggatgtgaactgagagtgaagttcagcaggagcgcagacgcccccgcgtaccagcagggccagaaccagctctataacgagctcaatctaggacgaagagaggagtacgatgttttggacaagagacgtggccgggaccctgagatggggggaaagccgagaaggaagaaccctcaggaaggcctgtacaatgaactgcagaaagataagatggcggaggcctacagtgagattgggatgaaaggcgagcgccggaggggcaaggggcacgatggcctttaccagggtctcagtacagccaccaaggacacctacgacgcccttcacatgcaggccctgccccctcgcgagggcagaggaagtcttctaacatgcggtgacgtggaggagaatcccggccctatgggggccgtcctgaggagcctcctggcctgcagcttctgtgtgctcctgagagcggagcagaaactcatctctgaagaggatctggaacctccaacatgttctcctcagcagtttacttgtttcacgggggaaattgactgtatccctgtggcttggcggtgcgatgggtttactgaatgtgaagaccacagtgatgaactcaattgtcctgtatgctcagagtcccagttccagtgtgccagtgggcagtgtattgatggtgccctccgatgcaatggagatgcaaactgccaggacaaatcagatgagaagaactgtgaagtgctttgtttaattgatcagttccgctgtgccaatggtcagtgcattggaaagcacaagaagtgtgatcataatgtggattgcagtgacaagtcagatgaactggattgttatccgactgaagaaccagcaccacaggccaccaatacagttggttctgttattggcgtaattgtcaccatttttgtgtctggaactgtatactttatctgccagaggatgttgtgtccacgtatgaagggagatggggaaactatgactaatgactatgtagttcatggaccagcttctgtgcctcttggttatgtgccacacccaagttctttgtcaggatctcttccaggaatgtctcgaggtaaatcaatgatcagctccctcagtatcatggggggaagcagtggacccccctatgaccgagcccatgttacaggagcatcatcaagtagttcttcaagcaccaaaggcacttacttccctgcaattttgaaccctccaccatccccagccacagagcgatcacattacactatggaatttggatattcttcaaacagtccttccactcataggtcatacagctacaggccatatagctaccggcactttgcaccccccaccacaccctgcagcacagatgtttgtgacagtgactatgctcctagtcggagaatgacctcagtggcaacagccaagggctataccagtgacttgaactatgattcagaacctgtgcccccacctcccacaccccgaagccaatacttgtcagcagaggagaactatgaaagctgcccaccttctccatacacagagaggagctattctcatcacctctacccaccgccaccctctccctgtacagactcctcctga

SEQ ID NO: 92 - protein, 781 aa, synthetic construct
  REGION 1..781: note = 4B3 VHH-ori2 CAR amino acid sequence
MALPVTALLLPLALLLHAARPEVQLVESGGGLVQPGGSLRLSCAASGLIFSRYVMGWFRQAPGKGRELVAFINSSGGSTNYPDSVEGRFTISRDNAKRMVYLQMNSLRAEDTAVYYCAASSRTSTTRGYNYWGQGTQVTVSSTTTPAPRPPTPAPTIASQPLSLRPEACRPAAGGAVHTRGLDFACDIYIWAPLAGTCGVLLLSLVITLYCKRGRKKLLYIFKQPFMRPVQTTQEEDGCSCRFPEEEEGGCELRVKFSRSADAPAYQQGQNQLYNELNLGRREEYDVLDKRRGRDPEMGGKPRRKNPQEGLYNELQKDKMAEAYSEIGMKGERRRGKGHDGLYQGLSTATKDTYDALHMQALPPREGRGSLLTCGDVEENPGPMGAVLRSLLACSFCVLLRAEQKLISEEDLEPPTCSPQQFTCFTGEIDCIPVAWRCDGFTECEDHSDELNCPVCSESQFQCASGQCIDGALRCNGDANCQDKSDEKNCEVLCLIDQFRCANGQCIGKHKKCDHNVDCSDKSDELDCYPTEEPAPQATNTVGSVIGVIVTIFVSGTVYFICQRMLCPRMKGDGETMTNDYVVHGPASVPLGYVPHPSSLSGSLPGMSRGKSMISSLSIMGGSSGPPYDRAHVTGASSSSSSSTKGTYFPAILNPPPSPATERSHYTMEFGYSSNSPSTHRSYSYRPYSYRHFAPPTTPCSTDVCDSDYAPSRRMTSVATAKGYTSDLNYDSEPVPPPPTPRSQYLSAEENYESCPPSPYTERSYSHHLYPPPPSPCTDSS

SEQ ID NO: 93 - protein, 25 aa, synthetic construct
  REGION 1..25: note = (G4S)5 linker
GGGGSGGGGSGGGGSGGGGSGGGGS

SEQ ID NO: 94 - protein, 20 aa, synthetic construct
  REGION 1..20: note = (G4S)4 linker
GGGGSGGGGSGGGGSGGGGS

SEQ ID NO: 95 - protein, 8 aa, synthetic construct
  REGION 1..8: note = 3B5 HCDR1
GFIFSRYG

SEQ ID NO: 96 - protein, 8 aa, synthetic construct
  REGION 1..8: note = 3B5 HCDR2
INWSDGTT

SEQ ID NO: 97 - protein, 14 aa, synthetic construct
  REGION 1..14: note = 3B5 HCDR3
AADRRLRSQTGYDY

SEQ ID NO: 98 - protein, 25 aa, synthetic construct [sequence omitted]

SEQ ID NO: 99 - protein, 17 aa, synthetic construct
  REGION 1..17: note = 3B5, 3E7, 3E9, 4A4, 4F10, 505A1, 505A11, 505D2, 505H3, 505H8, 505H10, 506A5, 506A8, 506B6, 506B12, 506C2, 506D2, 506D8, 506E1, 506F5, 506G1, 506H2, 506H9 FR2
MGWFRQAPGKGRELVAA

SEQ ID NO: 100 - protein, 38 aa, synthetic construct
  REGION 1..38: note = 3B5, 3E7, 4A2, 3E9, 3F5, 3G4, 4E12, 4F10, 505A1, 505A3, 505B12, 505D2, 505H3, 505H8, 505H10, 506A5, 506A8, 506B12, 506C2, 506C5, 506C8, 506C11, 506D8, 506E1, 506F5, 506G1, 506H2 FR3
YYPDSVEGRFTISRDNAKRMVYLQMNSLRAEDTAVYYC

SEQ ID NO: 101 - protein, 11 aa, synthetic construct
  REGION 1..11: note = FR4
WGQGTQVTVSS

SEQ ID NO: 102 - protein, 8 aa, synthetic construct
  REGION 1..8: note = 3E7 HCDR1
GRIFSRDA

SEQ ID NO: 103 - protein, 8 aa, synthetic construct
  REGION 1..8: note = 3E7 HCDR2
INSSGGNT

SEQ ID NO: 104 - protein, 17 aa, synthetic construct
  REGION 1..17: note = 3E7 HCDR3
AARGVRWTSTTAYGYNY

SEQ ID NO: 105 - protein, 8 aa, synthetic construct
  REGION 1..8: note = 4A2, 3E9 HCDR1
GFIFSRYD

SEQ ID NO: 106 - protein, 8 aa, synthetic construct
  REGION 1..8: note = 4A2, 506D8 HCDR2
ITWGGGST

SEQ ID NO: 107 - protein, 17 aa, synthetic construct
  REGION 1..17: note = 4A2 HCDR3
AARSASAYRTGRLEYNY

SEQ ID NO: 108 - protein, 17 aa, synthetic construct
  REGION 1..17: note = 4A2 H-FR2
MGWFRQAPGKGRELVAV

SEQ ID NO: 109 - protein, 8 aa, synthetic construct
  REGION 1..8: note = 4B3 HCDR1
GLIFSRYV

SEQ ID NO: 110 - protein, 8 aa, synthetic construct
  REGION 1..8: note = 4B3 HCDR2
INSSGGST

SEQ ID NO: 111 - protein, 14 aa, synthetic construct
  REGION 1..14: note = 4B3 HCDR3
AASSRTSTTRGYNY

SEQ ID NO: 112 - protein, 17 aa, synthetic construct
  REGION 1..17: note = 4B3, 3F5, 4E12 H-FR2
MGWFRQAPGKGRELVAF

SEQ ID NO: 113 - protein, 38 aa, synthetic construct
  REGION 1..38: note = 4B3, 506B6, 506H9 H-FR3
NYPDSVEGRFTISRDNAKRMVYLQMNSLRAEDTAVYYC

SEQ ID NO: 114 - protein, 8 aa, synthetic construct
  REGION 1..8: note = 3E9 HCDR2
INWGDSST

SEQ ID NO: 115 - protein, 17 aa, synthetic construct
  REGION 1..17: note = 3E9 HCDR3
AARRYYSYYPSSGGYNY

SEQ ID NO: 116 - protein, 8 aa, synthetic construct
  REGION 1..8: note = 3F5 HCDR1
GFILSRYV

SEQ ID NO: 117 - protein, 8 aa, synthetic construct
  REGION 1..8: note = 3F5 HCDR2
ITWSDGST

SEQ ID NO: 118 - protein, 14 aa, synthetic construct
  REGION 1..14: note = 3F5 HCDR3
AAKSRTYRGGLYDY

SEQ ID NO: 119 - protein, 8 aa, synthetic construct
  REGION 1..8: note = 3G4 HCDR1
GSIFSTYR

SEQ ID NO: 120 - protein, 8 aa, synthetic construct
  REGION 1..8: note = 3G4 HCDR2
ISPGGSDT

SEQ ID NO: 121 - protein, 17 aa, synthetic construct
  REGION 1..17: note = 3G4 HCDR3
AATPGRFALLSPRGYNY

SEQ ID NO: 122 - protein, 17 aa, synthetic construct
  REGION 1..17: note = 3G4, 505A3, 505B12H-FR2
MGWFRQAPGKGRELVAG

SEQ ID NO: 123 - protein, 8 aa, synthetic construct
  REGION 1..8: note = 4A4, 505H8 HCDR1
GFIFSRNA

SEQ ID NO: 124 - protein, 8 aa, synthetic construct
  REGION 1..8: note = 4A4 HCDR2
INWSGSST

SEQ ID NO: 125 - protein, 21 aa, synthetic construct
  REGION 1..21: note = 4A4 HCDR3
AAGSRTNTGTDWSRTRYTYNY

SEQ ID NO: 126 - protein, 38 aa, synthetic construct
  REGION 1..38: note = 4A4 H-FR3
FYPDSVEGRFTISRDNAKRMVYLQMNSLRAEDTAVYYC

SEQ ID NO: 127 - protein, 8 aa, synthetic construct
  REGION 1..8: note = 4E12 HCDR1
GFIFSRNS

SEQ ID NO: 128 - protein, 8 aa, synthetic construct
  REGION 1..8: note = 4E12 HCDR2
ISWRDGST

SEQ ID NO: 129 - protein, 14 aa, synthetic construct
  REGION 1..14: note = 4E12 HCDR3
AAFRGWNNGRNYNY

SEQ ID NO: 130 - protein, 8 aa, synthetic construct
  REGION 1..8: note = 4F10 HCDR1
GFIFSLNA

SEQ ID NO: 131 - protein, 8 aa, synthetic construct
  REGION 1..8: note = 4F10 HCDR2
ISPGDGTT

SEQ ID NO: 132 - protein, 14 aa, synthetic construct
  REGION 1..14: note = 4F10 HCDR3
AARRRSLSGYGYNY

SEQ ID NO: 133 - protein, 8 aa, synthetic construct
  REGION 1..8: note = 505A1 HCDR1
GYIFSRYN

SEQ ID NO: 134 - protein, 8 aa, synthetic construct
  REGION 1..8: note = 505A1, 505A3 HCDR2
ISAGGSST

SEQ ID NO: 135 - protein, 14 aa, synthetic construct
  REGION 1..14: note = 505A1 HCDR3
AARRRRATDSPYDY

SEQ ID NO: 136 - protein, 8 aa, synthetic construct
  REGION 1..8: note = 505A3 HCDR1
GFIFSRYS

SEQ ID NO: 137 - protein, 17 aa, synthetic construct
  REGION 1..17: note = 505A3 HCDR3
AAFARSPRTSTEYLYDY

SEQ ID NO: 138 - protein, 8 aa, synthetic construct
  REGION 1..8: note = 505A11 HCDR1
GIIFSRYV

SEQ ID NO: 139 - protein, 8 aa, synthetic construct
  REGION 1..8: note = 505A11 HCDR2
ITSGGGST

SEQ ID NO: 140 - protein, 17 aa, synthetic construct
  REGION 1..17: note = 505A11 HCDR3
AAGPRPNYGQRYNTYNY

SEQ ID NO: 141 - protein, 38 aa, synthetic construct
  REGION 1..38: note = 505A11, 505F1 FR3
HYPDSVEGRFTISRDNAKRMVYLQMNSLRAEDTAVYYC

SEQ ID NO: 142 - protein, 8 aa, synthetic construct
  REGION 1..8: note = 505B12 HCDR1
GFIFSRYI

SEQ ID NO: 143 - protein, 8 aa, synthetic construct
  REGION 1..8: note = 505B12 HCDR2
INAGGGST

SEQ ID NO: 144 - protein, 21 aa, synthetic construct
  REGION 1..21: note = 505B12 HCDR3
AAGSASGWSTYSPRRLYRYNY

SEQ ID NO: 145 - protein, 8 aa, synthetic construct
  REGION 1..8: note = 505D2 HCDR1
GYIFSRYA

SEQ ID NO: 146 - protein, 8 aa, synthetic construct
  REGION 1..8: note = 505D2 HCDR2
INRGGSTT

SEQ ID NO: 147 - protein, 14 aa, synthetic construct
  REGION 1..14: note = 505D2 HCDR3
AAGRFGLGSRTYDY

SEQ ID NO: 148 - protein, 8 aa, synthetic construct
  REGION 1..8: note = 505F1 HCDR1
GRTLSNNT

SEQ ID NO: 149 - protein, 8 aa, synthetic construct
  REGION 1..8: note = 505F1 HCDR2
ISASGSRT

SEQ ID NO: 150 - protein, 17 aa, synthetic construct
  REGION 1..17: note = 505F1 HCDR3
AAVSRVGFYTRGATYNY

SEQ ID NO: 151 - protein, 17 aa, synthetic construct
  REGION 1..17: note = 505F1, 506C8, 506C11 H-FR2
MGWFRQAPGKGRELVAS

SEQ ID NO: 152 - protein, 8 aa, synthetic construct
  REGION 1..8: note = 505H3 HCDR1
GNILSINI

SEQ ID NO: 153 - protein, 8 aa, synthetic construct
  REGION 1..8: note = 505H3, 505H10, 506C2 HCDR2
ISRTGGST

SEQ ID NO: 154 - protein, 14 aa, synthetic construct
  REGION 1..14: note = 505H3 HCDR3
AASSRRSSLNTYNY

SEQ ID NO: 155 - protein, 8 aa, synthetic construct
  REGION 1..8: note = 505H8 HCDR2
ITWSGGTT

SEQ ID NO: 156 - protein, 14 aa, synthetic construct
  REGION 1..14: note = 505H8 HCDR3
AARIAYSSTWTYDY

SEQ ID NO: 157 - protein, 8 aa, synthetic construct
  REGION 1..8: note = 505H10, 506C5 HCDR1
GFIFSRYY

SEQ ID NO: 158 - protein, 14 aa, synthetic construct
  REGION 1..14: note = 505H10 HCDR3
AADLYPGFRRGYNY

SEQ ID NO: 159 - protein, 8 aa, synthetic construct
  REGION 1..8: note = 506A5, 506A8, 506B6, 506G1HCDR1
GFIFSRYA

SEQ ID NO: 160 - protein, 8 aa, synthetic construct
  REGION 1..8: note = 506A5 HCDR2
ISRGDSDT

SEQ ID NO: 161 - protein, 17 aa, synthetic construct
  REGION 1..17: note = 506A5 HCDR3
AAVGRYYYGYYANNYNY

SEQ ID NO: 162 - protein, 8 aa, synthetic construct
  REGION 1..8: note = 506A8 HCDR2
INRGDSVT

SEQ ID NO: 163 - protein, 14 aa, synthetic construct
  REGION 1..14: note = 506A8 HCDR3
AARGRTSLAYTYDY

SEQ ID NO: 164 - protein, 8 aa, synthetic construct
  REGION 1..8: note = 506B6 HCDR2
INAGGGTT

SEQ ID NO: 165 - protein, 17 aa, synthetic construct
  REGION 1..17: note = 506B6 HCDR3
AAFTKRSLLTGSAVYNY

SEQ ID NO: 166 - protein, 8 aa, synthetic construct
  REGION 1..8: note = 506B12 HCDR1
GLIFSRNA

SEQ ID NO: 167 - protein, 8 aa, synthetic construct
  REGION 1..8: note = 506B12 HCDR2
INWGGGTT

SEQ ID NO: 168 - protein, 14 aa, synthetic construct
  REGION 1..14: note = 506B12 HCDR3
AATTRTSRPYTYNY

SEQ ID NO: 169 - protein, 8 aa, synthetic construct
  REGION 1..8: note = 506C2 CDR1
GYIFSNDV

SEQ ID NO: 170 - protein, 21 aa, synthetic construct
  REGION 1..21: note = 506C2 HCDR3
AASTRRRYATVDYRRDYTYDY

SEQ ID NO: 171 - protein, 8 aa, synthetic construct
  REGION 1..8: note = 506C5 HCDR2
ITSGDGST

SEQ ID NO: 172 - protein, 14 aa, synthetic construct
  REGION 1..14: note = 506C5 HCDR3
AARSFRRDIYDYNY

SEQ ID NO: 173 - protein, 17 aa, synthetic construct
  REGION 1..17: note = 506C5 H-FR2
MGWFRQAPGKGRELVAR

SEQ ID NO: 174 - protein, 8 aa, synthetic construct
  REGION 1..8: note = 506C8 HCDR1
GYIFSNYA

SEQ ID NO: 175 - protein, 8 aa, synthetic construct
  REGION 1..8: note = 506C8 HCDR2
INRSGSIT

SEQ ID NO: 176 - protein, 14 aa, synthetic construct
  REGION 1..14: note = 506C8 HCDR3
AANDVRGYYRRYNY

SEQ ID NO: 177 - protein, 8 aa, synthetic construct
  REGION 1..8: note = 506C11 HCDR1
GLIFSSYA

SEQ ID NO: 178 - protein, 8 aa, synthetic construct
  REGION 1..8: note = 506C11 HCDR2
INRRGGST

SEQ ID NO: 179 - protein, 14 aa, synthetic construct
  REGION 1..14: note = 506C11, 506G1 HCDR3
AAGSRSSSRLGYNY

SEQ ID NO: 180 - protein, 8 aa, synthetic construct
  REGION 1..8: note = 506D2 HCDR1
GIIFSRYA

SEQ ID NO: 181 - protein, 8 aa, synthetic construct
  REGION 1..8: note = 506D2 HCDR2
INRSGGRT

SEQ ID NO: 182 - protein, 14 aa, synthetic construct
  REGION 1..14: note = 506D2 HCDR3
AAFLASWDGTTYDY

SEQ ID NO: 183 - protein, 38 aa, synthetic construct
  REGION 1..38: note = 506D2 H-FR3
SYPDSVEGRFTISRDNAKRMVYLQMNSLRAEDTAVYYC

SEQ ID NO: 184 - protein, 8 aa, synthetic construct
  REGION 1..8: note = 506D8 HCDR1
GYTLSSYY

SEQ ID NO: 185 - protein, 21 aa, synthetic construct
  REGION 1..21: note = 506D8 HCDR3
AAARKRSVTYTTLSYAYSYDY

SEQ ID NO: 186 - protein, 8 aa, synthetic construct
  REGION 1..8: note = 506E1 HCDR1
GYIFSRYS

SEQ ID NO: 187 - protein, 8 aa, synthetic construct
  REGION 1..8: note = 506E1 HCDR2
ISSSGSST

SEQ ID NO: 188 - protein, 12 aa, synthetic construct
  REGION 1..12: note = 506E1 HCDR3
AATPRRSTGNTF

SEQ ID NO: 189 - protein, 8 aa, synthetic construct
  REGION 1..8: note = 506F5 HCDR1
GGIFSSYA

SEQ ID NO: 190 - protein, 8 aa, synthetic construct
  REGION 1..8: note = 506F5 HCDR2
INRGGGGT

SEQ ID NO: 191 - protein, 17 aa, synthetic construct
  REGION 1..17: note = 506F5 HCDR3
AAFGRYSRGSDDSRYNY

SEQ ID NO: 192 - protein, 8 aa, synthetic construct
  REGION 1..8: note = 506G1 HCDR2
ISWSGGST

SEQ ID NO: 193 - protein, 8 aa, synthetic construct
  REGION 1..8: note = 506H2 HCDR1
GRTFSYYT

SEQ ID NO: 194 - protein, 7 aa, synthetic construct
  REGION 1..7: note = 506H2 HCDR2
TSRDGST

SEQ ID NO: 195 - protein, 14 aa, synthetic construct
  REGION 1..14: note = 506H2 HCDR3
AAVRRWSSDSTYNY

SEQ ID NO: 196 - protein, 8 aa, synthetic construct
  REGION 1..8: note = 506H9 HCDR1
GRTFSRYA

SEQ ID NO: 197 - protein, 8 aa, synthetic construct
  REGION 1..8: note = 506H9 HCDR2
ISSRGSTT

SEQ ID NO: 198 - protein, 17 aa, synthetic construct
  REGION 1..17: note = 506H9 HCDR3
AASLYVIPAWNEYGYNY

SEQ ID NO: 199 - protein, 785 aa, synthetic construct
  REGION 1..785: note = 3E9 VHH-ori2 CAR amino acid sequence
  SITE 785: note = misc_feature - Xaa = any one kind of amino acid
MALPVTALLLPLALLLHAARPEVQLVESGGGLVQPGGSLRLSCAASGFIFSRYDMGWFRQAPGKGRELVAAINWGDSSTYYPDSVEGRFTISRDNAKRMVYLQMNSLRAEDTAVYYCAARRYYSYYPSSGGYNYWGQGTQVTVSSTTTPAPRPPTPAPTIASQPLSLRPEACRPAAGGAVHTRGLDFACDIYIWAPLAGTCGVLLLSLVITLYCKRGRKKLLYIFKQPFMRPVQTTQEEDGCSCRFPEEEEGGCELRVKFSRSADAPAYQQGQNQLYNELNLGRREEYDVLDKRRGRDPEMGGKPRRKNPQEGLYNELQKDKMAEAYSEIGMKGERRRGKGHDGLYQGLSTATKDTYDALHMQALPPREGRGSLLTCGDVEENPGPMGAVLRSLLACSFCVLLRAEQKLISEEDLEPPTCSPQQFTCFTGEIDCIPVAWRCDGFTECEDHSDELNCPVCSESQFQCASGQCIDGALRCNGDANCQDKSDEKNCEVLCLIDQFRCANGQCIGKHKKCDHNVDCSDKSDELDCYPTEEPAPQATNTVGSVIGVIVTIFVSGTVYFICQRMLCPRMKGDGETMTNDYVVHGPASVPLGYVPHPSSLSGSLPGMSRGKSMISSLSIMGGSSGPPYDRAHVTGASSSSSSSTKGTYFPAILNPPPSPATERSHYTMEFGYSSNSPSTHRSYSYRPYSYRHFAPPTTPCSTDVCDSDYAPSRRMTSVATAKGYTSDLNYDSEPVPPPPTPRSQYLSAEENYESCPPSPYTERSYSHHLYPPPPSPCTDSSX

SEQ ID NO: 200 - protein, 782 aa, synthetic construct
  REGION 1..782: note = 3F5 VHH-ori2 CAR amino acid sequence
  SITE 782: note = misc_feature - Xaa = any one kind of amino acid
MALPVTALLLPLALLLHAARPEVQLVESGGGLVQPGGSLRLSCAASGFILSRYVMGWFRQAPGKGRELVAFITWSDGSTYYPDSVEGRFTISRDNAKRMVYLQMNSLRAEDTAVYYCAAKSRTYRGGLYDYWGQGTQVTVSSTTTPAPRPPTPAPTIASQPLSLRPEACRPAAGGAVHTRGLDFACDIYIWAPLAGTCGVLLLSLVITLYCKRGRKKLLYIFKQPFMRPVQTTQEEDGCSCRFPEEEEGGCELRVKFSRSADAPAYQQGQNQLYNELNLGRREEYDVLDKRRGRDPEMGGKPRRKNPQEGLYNELQKDKMAEAYSEIGMKGERRRGKGHDGLYQGLSTATKDTYDALHMQALPPREGRGSLLTCGDVEENPGPMGAVLRSLLACSFCVLLRAEQKLISEEDLEPPTCSPQQFTCFTGEIDCIPVAWRCDGFTECEDHSDELNCPVCSESQFQCASGQCIDGALRCNGDANCQDKSDEKNCEVLCLIDQFRCANGQCIGKHKKCDHNVDCSDKSDELDCYPTEEPAPQATNTVGSVIGVIVTIFVSGTVYFICQRMLCPRMKGDGETMTNDYVVHGPASVPLGYVPHPSSLSGSLPGMSRGKSMISSLSIMGGSSGPPYDRAHVTGASSSSSSSTKGTYFPAILNPPPSPATERSHYTMEFGYSSNSPSTHRSYSYRPYSYRHFAPPTTPCSTDVCDSDYAPSRRMTSVATAKGYTSDLNYDSEPVPPPPTPRSQYLSAEENYESCPPSPYTERSYSHHLYPPPPSPCTDSSX

SEQ ID NO: 201 - protein, 785 aa, synthetic construct
  REGION 1..785: note = 3G4 VHH-ori2 CAR amino acid sequence
  SITE 785: note = misc_feature - Xaa = any one kind of amino acid
MALPVTALLLPLALLLHAARPEVQLVESGGGLVQPGGSLRLSCAASGSIFSTYRMGWFRQAPGKGRELVAGISPGGSDTYYPDSVEGRFTISRDNAKRMVYLQMNSLRAEDTAVYYCAATPGRFALLSPRGYNYWGQGTQVTVSSTTTPAPRPPTPAPTIASQPLSLRPEACRPAAGGAVHTRGLDFACDIYIWAPLAGTCGVLLLSLVITLYCKRGRKKLLYIFKQPFMRPVQTTQEEDGCSCRFPEEEEGGCELRVKFSRSADAPAYQQGQNQLYNELNLGRREEYDVLDKRRGRDPEMGGKPRRKNPQEGLYNELQKDKMAEAYSEIGMKGERRRGKGHDGLYQGLSTATKDTYDALHMQALPPREGRGSLLTCGDVEENPGPMGAVLRSLLACSFCVLLRAEQKLISEEDLEPPTCSPQQFTCFTGEIDCIPVAWRCDGFTECEDHSDELNCPVCSESQFQCASGQCIDGALRCNGDANCQDKSDEKNCEVLCLIDQFRCANGQCIGKHKKCDHNVDCSDKSDELDCYPTEEPAPQATNTVGSVIGVIVTIFVSGTVYFICQRMLCPRMKGDGETMTNDYVVHGPASVPLGYVPHPSSLSGSLPGMSRGKSMISSLSIMGGSSGPPYDRAHVTGASSSSSSSTKGTYFPAILNPPPSPATERSHYTMEFGYSSNSPSTHRSYSYRPYSYRHFAPPTTPCSTDVCDSDYAPSRRMTSVATAKGYTSDLNYDSEPVPPPPTPRSQYLSAEENYESCPPSPYTERSYSHHLYPPPPSPCTDSSX

SEQ ID NO: 202 - protein, 789 aa, synthetic construct
  REGION 1..789: note = 4A4 VHH-ori2 CAR amino acid sequence
  SITE 789: note = misc_feature - Xaa = any one kind of amino acid
MALPVTALLLPLALLLHAARPEVQLVESGGGLVQPGGSLRLSCAASGFIFSRNAMGWFRQAPGKGRELVAAINWSGSSTFYPDSVEGRFTISRDNAKRMVYLQMNSLRAEDTAVYYCAAGSRTNTGTDWSRTRYTYNYWGQGTQVTVSSTTTPAPRPPTPAPTIASQPLSLRPEACRPAAGGAVHTRGLDFACDIYIWAPLAGTCGVLLLSLVITLYCKRGRKKLLYIFKQPFMRPVQTTQEEDGCSCRFPEEEEGGCELRVKFSRSADAPAYQQGQNQLYNELNLGRREEYDVLDKRRGRDPEMGGKPRRKNPQEGLYNELQKDKMAEAYSEIGMKGERRRGKGHDGLYQGLSTATKDTYDALHMQALPPREGRGSLLTCGDVEENPGPMGAVLRSLLACSFCVLLRAEQKLISEEDLEPPTCSPQQFTCFTGEIDCIPVAWRCDGFTECEDHSDELNCPVCSESQFQCASGQCIDGALRCNGDANCQDKSDEKNCEVLCLIDQFRCANGQCIGKHKKCDHNVDCSDKSDELDCYPTEEPAPQATNTVGSVIGVIVTIFVSGTVYFICQRMLCPRMKGDGETMTNDYVVHGPASVPLGYVPHPSSLSGSLPGMSRGKSMISSLSIMGGSSGPPYDRAHVTGASSSSSSSTKGTYFPAILNPPPSPATERSHYTMEFGYSSNSPSTHRSYSYRPYSYRHFAPPTTPCSTDVCDSDYAPSRRMTSVATAKGYTSDLNYDSEPVPPPPTPRSQYLSAEENYESCPPSPYTERSYSHHLYPPPPSPCTDSSX

SEQ ID NO: 203 - protein, 782 aa, synthetic construct
  REGION 1..782: note = 4E12 VHH-ori2 CAR amino acid sequence
  SITE 782: note = misc_feature - Xaa = any one kind of amino acid
MALPVTALLLPLALLLHAARPEVQLVESGGGLVQPGGSLRLSCAASGFIFSRNSMGWFRQAPGKGRELVAFISWRDGSTYYPDSVEGRFTISRDNAKRMVYLQMNSLRAEDTAVYYCAAFRGWNNGRNYNYWGQGTQVTVSSTTTPAPRPPTPAPTIASQPLSLRPEACRPAAGGAVHTRGLDFACDIYIWAPLAGTCGVLLLSLVITLYCKRGRKKLLYIFKQPFMRPVQTTQEEDGCSCRFPEEEEGGCELRVKFSRSADAPAYQQGQNQLYNELNLGRREEYDVLDKRRGRDPEMGGKPRRKNPQEGLYNELQKDKMAEAYSEIGMKGERRRGKGHDGLYQGLSTATKDTYDALHMQALPPREGRGSLLTCGDVEENPGPMGAVLRSLLACSFCVLLRAEQKLISEEDLEPPTCSPQQFTCFTGEIDCIPVAWRCDGFTECEDHSDELNCPVCSESQFQCASGQCIDGALRCNGDANCQDKSDEKNCEVLCLIDQFRCANGQCIGKHKKCDHNVDCSDKSDELDCYPTEEPAPQATNTVGSVIGVIVTIFVSGTVYFICQRMLCPRMKGDGETMTNDYVVHGPASVPLGYVPHPSSLSGSLPGMSRGKSMISSLSIMGGSSGPPYDRAHVTGASSSSSSSTKGTYFPAILNPPPSPATERSHYTMEFGYSSNSPSTHRSYSYRPYSYRHFAPPTTPCSTDVCDSDYAPSRRMTSVATAKGYTSDLNYDSEPVPPPPTPRSQYLSAEENYESCPPSPYTERSYSHHLYPPPPSPCTDSSX

SEQ ID NO: 204 - protein, 782 aa, synthetic construct
  REGION 1..782: note = 4F10 VHH-ori2 CAR amino acid sequence
  SITE 782: note = misc_feature - Xaa = any one kind of amino acid
MALPVTALLLPLALLLHAARPEVQLVESGGGLVQPGGSLRLSCAASGFIFSLNAMGWFRQAPGKGRELVAAISPGDGTTYYPDSVEGRFTISRDNAKRMVYLQMNSLRAEDTAVYYCAARRRSLSGYGYNYWGQGTQVTVSSTTTPAPRPPTPAPTIASQPLSLRPEACRPAAGGAVHTRGLDFACDIYIWAPLAGTCGVLLLSLVITLYCKRGRKKLLYIFKQPFMRPVQTTQEEDGCSCRFPEEEEGGCELRVKFSRSADAPAYQQGQNQLYNELNLGRREEYDVLDKRRGRDPEMGGKPRRKNPQEGLYNELQKDKMAEAYSEIGMKGERRRGKGHDGLYQGLSTATKDTYDALHMQALPPREGRGSLLTCGDVEENPGPMGAVLRSLLACSFCVLLRAEQKLISEEDLEPPTCSPQQFTCFTGEIDCIPVAWRCDGFTECEDHSDELNCPVCSESQFQCASGQCIDGALRCNGDANCQDKSDEKNCEVLCLIDQFRCANGQCIGKHKKCDHNVDCSDKSDELDCYPTEEPAPQATNTVGSVIGVIVTIFVSGTVYFICQRMLCPRMKGDGETMTNDYVVHGPASVPLGYVPHPSSLSGSLPGMSRGKSMISSLSIMGGSSGPPYDRAHVTGASSSSSSSTKGTYFPAILNPPPSPATERSHYTMEFGYSSNSPSTHRSYSYRPYSYRHFAPPTTPCSTDVCDSDYAPSRRMTSVATAKGYTSDLNYDSEPVPPPPTPRSQYLSAEENYESCPPSPYTERSYSHHLYPPPPSPCTDSSX

SEQ ID NO: 205 - protein, 365 aa, synthetic construct
  REGION 1..365: note = 3B5 VHH CAR amino acid sequence
MALPVTALLLPLALLLHAARPEVQLVESGGGLVQPGGSLRLSCAASGFIFSRYGMGWFRQAPGKGRELVAAINWSDGTTYYPDSVEGRFTISRDNAKRMVYLQMNSLRAEDTAVYYCAADRRLRSQTGYDYWGQGTQVTVSSTTTPAPRPPTPAPTIASQPLSLRPEACRPAAGGAVHTRGLDFACDIYIWAPLAGTCGVLLLSLVITLYCKRGRKKLLYIFKQPFMRPVQTTQEEDGCSCRFPEEEEGGCELRVKFSRSADAPAYQQGQNQLYNELNLGRREEYDVLDKRRGRDPEMGGKPRRKNPQEGLYNELQKDKMAEAYSEIGMKGERRRGKGHDGLYQGLSTATKDTYDALHMQALPPR

SEQ ID NO: 206 - protein, 368 aa, synthetic construct
  REGION 1..368: note = 3E7 VHH CAR amino acid sequence
MALPVTALLLPLALLLHAARPEVQLVESGGGLVQPGGSLRLSCAASGRIFSRDAMGWFRQAPGKGRELVAAINSSGGNTYYPDSVEGRFTISRDNAKRMVYLQMNSLRAEDTAVYYCAARGVRWTSTTAYGYNYWGQGTQVTVSSTTTPAPRPPTPAPTIASQPLSLRPEACRPAAGGAVHTRGLDFACDIYIWAPLAGTCGVLLLSLVITLYCKRGRKKLLYIFKQPFMRPVQTTQEEDGCSCRFPEEEEGGCELRVKFSRSADAPAYQQGQNQLYNELNLGRREEYDVLDKRRGRDPEMGGKPRRKNPQEGLYNELQKDKMAEAYSEIGMKGERRRGKGHDGLYQGLSTATKDTYDALHMQALPPR

SEQ ID NO: 207 - protein, 368 aa, synthetic construct
  REGION 1..368: note = 4A2 VHH CAR amino acid sequence
MALPVTALLLPLALLLHAARPEVQLVESGGGLVQPGGSLRLSCAASGFIFSRYDMGWFRQAPGKGRELVAVITWGGGSTYYPDSVEGRFTISRDNAKRMVYLQMNSLRAEDTAVYYCAARSASAYRTGRLEYNYWGQGTQVTVSSTTTPAPRPPTPAPTIASQPLSLRPEACRPAAGGAVHTRGLDFACDIYIWAPLAGTCGVLLLSLVITLYCKRGRKKLLYIFKQPFMRPVQTTQEEDGCSCRFPEEEEGGCELRVKFSRSADAPAYQQGQNQLYNELNLGRREEYDVLDKRRGRDPEMGGKPRRKNPQEGLYNELQKDKMAEAYSEIGMKGERRRGKGHDGLYQGLSTATKDTYDALHMQALPPR

SEQ ID NO: 208 - protein, 365 aa, synthetic construct
  REGION 1..365: note = 4B3 VHH CAR amino acid sequence
MALPVTALLLPLALLLHAARPEVQLVESGGGLVQPGGSLRLSCAASGLIFSRYVMGWFRQAPGKGRELVAFINSSGGSTNYPDSVEGRFTISRDNAKRMVYLQMNSLRAEDTAVYYCAASSRTSTTRGYNYWGQGTQVTVSSTTTPAPRPPTPAPTIASQPLSLRPEACRPAAGGAVHTRGLDFACDIYIWAPLAGTCGVLLLSLVITLYCKRGRKKLLYIFKQPFMRPVQTTQEEDGCSCRFPEEEEGGCELRVKFSRSADAPAYQQGQNQLYNELNLGRREEYDVLDKRRGRDPEMGGKPRRKNPQEGLYNELQKDKMAEAYSEIGMKGERRRGKGHDGLYQGLSTATKDTYDALHMQALPPR

SEQ ID NO: 209 - protein, 368 aa, synthetic construct
  REGION 1..368: note = 3E9 VHH CAR amino acid sequence
MALPVTALLLPLALLLHAARPEVQLVESGGGLVQPGGSLRLSCAASGFIFSRYDMGWFRQAPGKGRELVAAINWGDSSTYYPDSVEGRFTISRDNAKRMVYLQMNSLRAEDTAVYYCAARRYYSYYPSSGGYNYWGQGTQVTVSSTTTPAPRPPTPAPTIASQPLSLRPEACRPAAGGAVHTRGLDFACDIYIWAPLAGTCGVLLLSLVITLYCKRGRKKLLYIFKQPFMRPVQTTQEEDGCSCRFPEEEEGGCELRVKFSRSADAPAYQQGQNQLYNELNLGRREEYDVLDKRRGRDPEMGGKPRRKNPQEGLYNELQKDKMAEAYSEIGMKGERRRGKGHDGLYQGLSTATKDTYDALHMQALPPR

SEQ ID NO: 210 - protein, 365 aa, synthetic construct
  REGION 1..365: note = 3F5 VHH CAR amino acid sequence
MALPVTALLLPLALLLHAARPEVQLVESGGGLVQPGGSLRLSCAASGFILSRYVMGWFRQAPGKGRELVAFITWSDGSTYYPDSVEGRFTISRDNAKRMVYLQMNSLRAEDTAVYYCAAKSRTYRGGLYDYWGQGTQVTVSSTTTPAPRPPTPAPTIASQPLSLRPEACRPAAGGAVHTRGLDFACDIYIWAPLAGTCGVLLLSLVITLYCKRGRKKLLYIFKQPFMRPVQTTQEEDGCSCRFPEEEEGGCELRVKFSRSADAPAYQQGQNQLYNELNLGRREEYDVLDKRRGRDPEMGGKPRRKNPQEGLYNELQKDKMAEAYSEIGMKGERRRGKGHDGLYQGLSTATKDTYDALHMQALPPR

SEQ ID NO: 211 - protein, 368 aa, synthetic construct
  REGION 1..368: note = 3G4 VHH CAR amino acid sequence
MALPVTALLLPLALLLHAARPEVQLVESGGGLVQPGGSLRLSCAASGSIFSTYRMGWFRQAPGKGRELVAGISPGGSDTYYPDSVEGRFTISRDNAKRMVYLQMNSLRAEDTAVYYCAATPGRFALLSPRGYNYWGQGTQVTVSSTTTPAPRPPTPAPTIASQPLSLRPEACRPAAGGAVHTRGLDFACDIYIWAPLAGTCGVLLLSLVITLYCKRGRKKLLYIFKQPFMRPVQTTQEEDGCSCRFPEEEEGGCELRVKFSRSADAPAYQQGQNQLYNELNLGRREEYDVLDKRRGRDPEMGGKPRRKNPQEGLYNELQKDKMAEAYSEIGMKGERRRGKGHDGLYQGLSTATKDTYDALHMQALPPR

SEQ ID NO: 212 - protein, 372 aa, synthetic construct
  REGION 1..372: note = 4A4 VHH CAR amino acid sequence
MALPVTALLLPLALLLHAARPEVQLVESGGGLVQPGGSLRLSCAASGFIFSRNAMGWFRQAPGKGRELVAAINWSGSSTFYPDSVEGRFTISRDNAKRMVYLQMNSLRAEDTAVYYCAAGSRTNTGTDWSRTRYTYNYWGQGTQVTVSSTTTPAPRPPTPAPTIASQPLSLRPEACRPAAGGAVHTRGLDFACDIYIWAPLAGTCGVLLLSLVITLYCKRGRKKLLYIFKQPFMRPVQTTQEEDGCSCRFPEEEEGGCELRVKFSRSADAPAYQQGQNQLYNELNLGRREEYDVLDKRRGRDPEMGGKPRRKNPQEGLYNELQKDKMAEAYSEIGMKGERRRGKGHDGLYQGLSTATKDTYDALHMQALPPR

SEQ ID NO: 213 - protein, 365 aa, synthetic construct
  REGION 1..365: note = 4E12 VHH CAR amino acid sequence
MALPVTALLLPLALLLHAARPEVQLVESGGGLVQPGGSLRLSCAASGFIFSRNSMGWFRQAPGKGRELVAFISWRDGSTYYPDSVEGRFTISRDNAKRMVYLQMNSLRAEDTAVYYCAAFRGWNNGRNYNYWGQGTQVTVSSTTTPAPRPPTPAPTIASQPLSLRPEACRPAAGGAVHTRGLDFACDIYIWAPLAGTCGVLLLSLVITLYCKRGRKKLLYIFKQPFMRPVQTTQEEDGCSCRFPEEEEGGCELRVKFSRSADAPAYQQGQNQLYNELNLGRREEYDVLDKRRGRDPEMGGKPRRKNPQEGLYNELQKDKMAEAYSEIGMKGERRRGKGHDGLYQGLSTATKDTYDALHMQALPPR

SEQ ID NO: 214 - protein, 365 aa, synthetic construct
  REGION 1..365: note = 4F10 VHH CAR amino acid sequence
MALPVTALLLPLALLLHAARPEVQLVESGGGLVQPGGSLRLSCAASGFIFSLNAMGWFRQAPGKGRELVAAISPGDGTTYYPDSVEGRFTISRDNAKRMVYLQMNSLRAEDTAVYYCAARRRSLSGYGYNYWGQGTQVTVSSTTTPAPRPPTPAPTIASQPLSLRPEACRPAAGGAVHTRGLDFACDIYIWAPLAGTCGVLLLSLVITLYCKRGRKKLLYIFKQPFMRPVQTTQEEDGCSCRFPEEEEGGCELRVKFSRSADAPAYQQGQNQLYNELNLGRREEYDVLDKRRGRDPEMGGKPRRKNPQEGLYNELQKDKMAEAYSEIGMKGERRRGKGHDGLYQGLSTATKDTYDALHMQALPPR

SEQ ID NO: 215 - protein, 17 aa, synthetic construct
  REGION 1..17: note = 3E7 HCDR3; 4A2 HCDR3; 3E9 HCDR3; 3G4 HCDR3; 505A3 HCDR3; 505A11 HCDR3; 505F1 HCDR3; 506A5 HCDR3; 506B6 HCDR3; 506F5 HCDR3; 506H9 HCDR3 general formula
  SITE 3: note = misc_feature - Xaa = Phe, Gly, Arg, Ser, Thr or Val
  SITE 4: note = misc_feature - Xaa = Ala, Gly, Leu, Pro, Arg, Ser or Thr
  SITE 5: note = misc_feature - Xaa = Ala, Gly, Lys, Arg, Val or Tyr
  SITE 6: note = misc_feature - Xaa = Pro, Arg, Ser, Val or Tyr
  SITE 7: note = misc_feature - Xaa = Ala, Phe, Gly, Ile, Asn, Pro, Ser, Trp or Tyr
  SITE 8: note = misc_feature - Xaa = Ala, Phe, Leu, Pro, Arg, Thr or Tyr
  SITE 9: note = misc_feature - Xaa = Ala, Gly, Leu, Arg, Ser, Thr or Tyr
  SITE 10: note = misc_feature - Xaa = Leu, Pro, Gln, Ser, Thr, Trp or Tyr
  SITE 11: note = misc_feature - Xaa = Asp, Gly, Asn, Arg, Ser, Thr or Tyr
  SITE 12: note = misc_feature - Xaa = Ala, Asp, Glu, Gly, Pro, Arg, Ser or Tyr
  SITE 13: note = misc_feature - Xaa = Ala, Gly, Leu, Asn, Arg, Ser or Tyr
  SITE 14: note = misc_feature - Xaa = Glu, Gly, Leu, Asn, Arg, Thr or Val
  SITE 16: note = misc_feature - Xaa = Asp or Asn
AAXXXXXXXXXXXXYXY

SEQ ID NO: 216 - protein, 17 aa, synthetic construct
  REGION 1..17: note = H-FR2 general formula
  SITE 17: note = misc_feature - Xaa = Ala, Phe, Gly, Arg, Ser or Val
MGWFRQAPGKGRELVAX

SEQ ID NO: 217 - protein, 38 aa, synthetic construct
  REGION 1..38: note = H-FR3 general formula
  SITE 1: note = misc_feature - Xaa = Phe, His, Asn, Ser or Tyr
XYPDSVEGRFTISRDNAKRMVYLQMNSLRAEDTAVYYC

SEQ ID NO: 218 - protein, 14 aa, synthetic construct
  REGION 1..14: note = 3B5 HCDR3; 4B3 HCDR3; 3F5 HCDR3; 4E12 HCDR3; 505A1 HCDR3; 505H3 HCDR3; 505H8 HCDR3; 505H10 HCDR3; 506A8 HCDR3; 506C5 HCDR3; 506C8 HCDR3; 506C11 HCDR3; 506G1 HCDR3; 506D2 HCDR3 general formula
  SITE 3: note = misc_feature - Xaa = Asp, Phe, Gly, Lys, Asn, Arg or Ser
  SITE 4: note = misc_feature - Xaa = Asp, Gly, Ile, Leu, Arg or Ser
  SITE 5: note = misc_feature - Xaa = Ala, Phe, Gly, Arg, Val or Tyr
  SITE 6: note = misc_feature - Xaa = Leu, Pro, Arg, Ser, Thr, Trp or Tyr
  SITE 7: note = misc_feature - Xaa = Ala, Gly, Asn, Arg, Ser, Trp or Tyr
  SITE 8: note = misc_feature - Xaa = Asp, Phe, Leu, Asn, Arg, Ser, Thr or Tyr
  SITE 9: note = misc_feature - Xaa = Ala, Asp, Gly, Ile, Leu, Gln, Arg, Thr or Tyr
  SITE 10: note = misc_feature - Xaa = Gly, Leu, Asn, Arg, Ser, Thr, Trp or Tyr
  SITE 11: note = misc_feature - Xaa = Asp, Gly, Leu, Asn, Pro, Arg or Thr
  SITE 13: note = misc_feature - Xaa = Asp or Asn
AAXXXXXXXXXYXY

SEQ ID NO: 219-220 - skipped (2 entries)